European Patent Application EP 4 549 573 A1, published May 7, 2025. Title: PEPTIDE LINKER FOR LOCALIZING TRANSMEMBRANE PROTEIN TO TARGET ORGANELLE, LOCALIZATION METHOD THEREBY, AND LOCALIZED FUSION PROTEIN THEREWITH. Applicant: 浜松ホトニクス株式会社. The sequence listing filed with the application follows.

SEQUENCE LISTING (42 sequences)

SEQ ID NO: 1 - protein, 24 aa, synthetic construct
MLSLRQSIRFFKPATRTLCSSRYL

SEQ ID NO: 2 - protein, 140 aa, synthetic construct
MRAPSARALLLIPRRGPAVRAWAPAVSSRIWLASEWTPLVRAWTSLIHKPGSGLRFPAPLSGLPGGVGQWATSSGARRCWVLAGPRAAHPLFARLQGAAATGVRDLGNDSQRRPAATGRSEVWKLLGLVRPERGRLSAAV

SEQ ID NO: 3 - protein, 119 aa, synthetic construct
MALLRAAVSELRRRGRGALTPLPALSSLLSSLSPRSPASTRPEPNNPHADRRHVIALRRCPPLPASAVLAPELLHARGLLPRHWSHASPLSTSSSSSRPADKAQLTWVDKWIPEAARPY

SEQ ID NO: 4 - protein, 7 aa, synthetic construct
PKKKRRV

SEQ ID NO: 5 - protein, 5 aa, synthetic construct
EAAAK

SEQ ID NO: 6 - protein, 5 aa, synthetic construct
EAAAR

SEQ ID NO: 7 - protein, 5 aa, synthetic construct
EAAAQ

SEQ ID NO: 8 - protein, 5 aa, synthetic construct
DAAAK

SEQ ID NO: 9 - protein, 5 aa, synthetic construct
DAAAR

SEQ ID NO: 10 - protein, 5 aa, synthetic construct
DAAAQ

SEQ ID NO: 11 - protein, 583 aa, Mus musculus
RGRLSAAVGFLAVSSVITMSAPFFLGRIIDVIYTNPSEGYGDSLTRLCAVLTCVFLCGAAANGIRVYLMQSSGQSIVNRLRTSLFSSILRQEVAFFDKTRTGELINRLSSDTALLGRSVTENLSDGLRAGAQASVGVGMMFFVSPSLATFVLSVVPPISVLAVIYGRYLRKLSKATQDSLAEATQLAEERIGNIRTIRAFGKEMTEVEKYTGRVDQLLQLAQKEALARAGFFGAAGLSGNLIVLSVLYKGGLLMGSAHMTVGELSSFLMYAFWVGLSIGGLSSFYSELMKGLGAGGRLWELLERQPRLPFNEGMVLDEKTFQGALEFRNVHFTYPARPEVSVFQDFSLSIPSGSVTALVGPSGSGKSTVVSLLLRLYDPNSGTVSLDGHDIRQLNPVWLRSKIGTVSQEPVLFSCSVAENIAYGADNLSSVTAQQVERAAEVANAAEFIRSFPQGFDTVVGEKGILLSGGQKQRIAIARALLKNPKILLLDEATSALDAENEHLVQEALDRLMEGRTVLIIAHRLSTIKNANFVAVLDHGKICEHGTHEELLLKPNGLYRKLMNKQSFLSYNGAEQFLEPARA

SEQ ID NO: 12 - protein, 14 aa, synthetic construct
PAPAPAPAPAPAPP

SEQ ID NO: 13 - protein, 232 aa, synthetic construct
SSGTKLFTKEIPYVTELEGDVNGMKFTIHGKGTGDASTGTIKAKYICTTGDLPVPWATLVSTLSYGVQCFAKYPPEIKDFFKSAMPEGYVQERTITFEGDGVFKTRAEVTFENGSVYNRVTLTGQGFKKDGHILRKNVAFQCPPDIVYILPDTVNNGIRVEFNQAYDIEGVTEKLVTKCSQMNRPLAGSAAVHIPRYHHLSKHTKLSKDRDERRDHMCLVEVVKAVDLDTYQ

SEQ ID NO: 14 - protein, 966 aa, synthetic construct
MSVLTPLLLRGLTGSARRLPVPRAKGSAGSAPEPNPNPKPKPAPKPAPKPEPAPKPEPAPAPKPAPKPAPEPAPAPEPKPAPKPEPAPEPEPAPAPEPAPKPEPAPKPAPKPAPAPAPAPAPEPAPNPNPERGRLSAAVGFLAVSSVITMSAPFFLGRIIDVIYTNPSEGYGDSLTRLCAVLTCVFLCGAAANGIRVYLMQSSGQSIVNRLRTSLFSSILRQEVAFFDKTRTGELINRLSSDTALLGRSVTENLSDGLRAGAQASVGVGMMFFVSPSLATFVLSVVPPISVLAVIYGRYLRKLSKATQDSLAEATQLAEERIGNIRTIRAFGKEMTEVEKYTGRVDQLLQLAQKEALARAGFFGAAGLSGNLIVLSVLYKGGLLMGSAHMTVGELSSFLMYAFWVGLSIGGLSSFYSELMKGLGAGGRLWELLERQPRLPFNEGMVLDEKTFQGALEFRNVHFTYPARPEVSVFQDFSLSIPSGSVTALVGPSGSGKSTVVSLLLRLYDPNSGTVSLDGHDIRQLNPVWLRSKIGTVSQEPVLFSCSVAENIAYGADNLSSVTAQQVERAAEVANAAEFIRSFPQGFDTVVGEKGILLSGGQKQRIAIARALLKNPKILLLDEATSALDAENEHLVQEALDRLMEGRTVLIIAHRLSTIKNANFVAVLDHGKICEHGTHEELLLKPNGLYRKLMNKQSFLSYNGAEQFLEPARAPAPAPAPAPAPAPPSSGTKLFTKEIPYVTELEGDVNGMKFTIHGKGTGDASTGTIKAKYICTTGDLPVPWATLVSTLSYGVQCFAKYPPEIKDFFKSAMPEGYVQERTITFEGDGVFKTRAEVTFENGSVYNRVTLTGQGFKKDGHILRKNVAFQCPPDIVYILPDTVNNGIRVEFNQAYDIEGVTEKLVTKCSQMNRPLAGSAAVHIPRYHHLSKHTKLSKDRDERRDHMCLVEVVKAVDLDTYQHHHHHH

SEQ ID NO: 15 - DNA, 2898 bp, synthetic construct
  source 1..2898: mol_type = other DNA
atgtccgtcctgacgccgctgctgctgcggggcttgacaggctcggcccggcggctcccagtgccgcgcgccaagggatcagctggctctgcaccagagcctaatcccaatccaaagcctaagcctgcacctaaacctgctcctaaacctgaaccagctcctaagcctgaacctgctcctgcacccaaaccagctccaaaaccagcaccagaaccagctccagctcctgaacctaagcctgccccaaaaccagaacccgcacctgaacctgagcctgcaccagctccagagccagcccctaaacccgagccagcacctaagccagctcctaagccagccccagcacctgccccagcccccgcaccagaacctgcaccaaaccctaatcctgagcgcgggagactgtcagctgcagttgggtttctggctgtgtccagtgtcatcaccatgtctgcccccttcttcctgggaaggatcattgatgtcatctataccaacccaagcgagggctatggcgatagcttgactcggctctgtgctgtgctcacctgtgtgttcctgtgcggcgctgctgccaacggcattcgtgtctacctcatgcagtcttcaggtcagagcattgtgaacaggctgcgcacctctctgttctcctccattctaaggcaagaggttgctttctttgacaagacccgcacaggcgaattaattaaccgcctctcctcggataccgcactcctggggcgctccgtgactgagaacctctccgatggcctgagagctggggcccaggcctccgttggtgttggcatgatgttttttgtgtcaccaagtctggccacctttgttctgagtgtggtacctcccatctctgtcctcgctgtgatttatgggcgatatctacggaaactgtccaaagccacacaggactccttggcagaagccacacagctagccgaggagcggattggaaacataagaaccatccgagcttttgggaaggagatgacggaagtggagaagtacaccggccgagtggaccagttgctgcagctggcacagaaggaggccttggcacgagccggcttctttggagcagctgggctctcaggaaacctgattgtgctgtctgtcctgtacaaaggaggcctgctgatgggcagtgcccatatgacagtgggcgagctctcttccttcctcatgtacgctttctgggttggattgagcatcggaggactgagttcattctactccgagctgatgaaaggcctgggtgctggtgggcggctctgggagctgctggagagacagccacggctgccttttaacgaggggatggtgttagatgagaaaaccttccagggtgccctggagttcagaaacgtgcacttcacataccctgctcgcccagaggtgtccgtattccaggatttcagtctttccatcccgtctggatctgtcacagcgctggttggcccaagtggttctgggaaatcaacagtggtttcgctcctgctgcggttgtacgaccctaattctggaacagtcagccttgatggccatgacattcgtcagctaaaccccgtctggctgagatccaagattgggacagtgagtcaggagccagtcctgttctcctgctctgtcgctgagaacattgcctatggagctgacaacctctcctcggtcacagcccagcaggtggagagggccgcagaggtggccaacgctgctgagttcatccgaagcttcccacagggcttcgacactgtggtcggggagaagggcatcctcctgtccggtgggcagaagcagaggattgcaatagccagagccctgctgaagaaccccaaaattcttctccttgatgaagcaaccagtgcactggatgccgaaaatgagcacctggtccaggaggcgcttgaccggctgatggaagggagaactgtgctgatcatagcccaccgcctgtccaccattaagaatgccaactttgttgctgtccttgaccacggaaagatctgtgaacacgggacacatgaagagctgctcctgaagcccaatgggctttacagaaaactgatgaacaagcagagtttcctgtcatataatggagcagagcagttcctggaacctgcacgggcgcctgctcccgcaccagcccctgctcctgcaccagcacctcccagctccggtactaaactcttcaccaaggaaatcccctatgtgaccgagctggagggggacgtaaacggcatgaagtttactatccatggaaagggtaccggtgacgccagcaccgggacaatcaaagcgaaatacatctgcaccaccggcgatctaccggtgccctgggccactcttgtgagcaccctgtcctatggcgtccagtgcttcgcaaagtacccaccggaaatcaaggacttcttcaaatctgccatgccggagggctacgtacaagagaggactatcaccttcgagggcgatggtgtgttcaaaacgcgtgcagaggtcacttttgaaaatggttccgtctacaaccgagtcacgctgacgggccagggattcaaaaaggacggacatatcttgcgtaagaacgtcgcattccagtgtcccccagacatcgtgtacatcctgcccgacactgtgaataacggtatcagagtggagttcaaccaggcatacgatatcgaaggagtaactgagaagctggtgacaaaatgcagccagatgaaccggcctctcgctggctcagcggcagtccacatcccacgctaccaccacctgtcgaaacacaccaaactgtctaaagatcgggacgagaggagagatcatatgtgtctcgtggaggtggtgaaagcggtggacctcgatacgtaccagcaccaccatcaccatcat

SEQ ID NO: 16 - protein, 100 aa, synthetic construct
PEPNPNPKPKPAPKPAPKPEPAPKPEPAPAPKPAPKPAPEPAPAPEPKPAPKPEPAPEPEPAPAPEPAPKPEPAPKPAPKPAPAPAPAPAPEPAPNPNPE

SEQ ID NO: 17 - protein, 966 aa, synthetic construct
MSVLTPLLLRGLTGSARRLPVPRAKGSAGSAPKAPSKSPAAPKKKPAKPKKAPKKPKAAPKKPAAEPKAPAEAPAAPEAAPAEPAAAPEAPAAEPAAPAEAPAAPEAAPAEPAAAPEAPAAAPAAPSASPARGRLSAAVGFLAVSSVITMSAPFFLGRIIDVIYTNPSEGYGDSLTRLCAVLTCVFLCGAAANGIRVYLMQSSGQSIVNRLRTSLFSSILRQEVAFFDKTRTGELINRLSSDTALLGRSVTENLSDGLRAGAQASVGVGMMFFVSPSLATFVLSVVPPISVLAVIYGRYLRKLSKATQDSLAEATQLAEERIGNIRTIRAFGKEMTEVEKYTGRVDQLLQLAQKEALARAGFFGAAGLSGNLIVLSVLYKGGLLMGSAHMTVGELSSFLMYAFWVGLSIGGLSSFYSELMKGLGAGGRLWELLERQPRLPFNEGMVLDEKTFQGALEFRNVHFTYPARPEVSVFQDFSLSIPSGSVTALVGPSGSGKSTVVSLLLRLYDPNSGTVSLDGHDIRQLNPVWLRSKIGTVSQEPVLFSCSVAENIAYGADNLSSVTAQQVERAAEVANAAEFIRSFPQGFDTVVGEKGILLSGGQKQRIAIARALLKNPKILLLDEATSALDAENEHLVQEALDRLMEGRTVLIIAHRLSTIKNANFVAVLDHGKICEHGTHEELLLKPNGLYRKLMNKQSFLSYNGAEQFLEPARAPAPAPAPAPAPAPPSSGTKLFTKEIPYVTELEGDVNGMKFTIHGKGTGDASTGTIKAKYICTTGDLPVPWATLVSTLSYGVQCFAKYPPEIKDFFKSAMPEGYVQERTITFEGDGVFKTRAEVTFENGSVYNRVTLTGQGFKKDGHILRKNVAFQCPPDIVYILPDTVNNGIRVEFNQAYDIEGVTEKLVTKCSQMNRPLAGSAAVHIPRYHHLSKHTKLSKDRDERRDHMCLVEVVKAVDLDTYQHHHHHH

SEQ ID NO: 18 - DNA, 2898 bp, synthetic construct
  source 1..2898: mol_type = other DNA
atgtccgtcctgacgccgctgctgctgcggggcttgacaggctcggcccggcggctcccagtgccgcgcgccaagggatcagctggctctgcacctaaggccccatctaagtccccagccgctccaaagaagaagccagctaagcctaagaaggcacctaagaagccaaaggcagcaccaaagaagcctgcagcagaacctaaggcaccagcagaagcaccagcagcaccagaagcagctccagcagaaccagcagctgccccagaagcaccagctgccgagccagcagctcctgccgaggctcctgctgcccctgaggctgcacctgccgagcctgctgcagcccctgaggctcctgcagccgctcctgctgcaccaagtgcttctccagcacgcgggagactgtcagctgcagttgggtttctggctgtgtccagtgtcatcaccatgtctgcccccttcttcctgggaaggatcattgatgtcatctataccaacccaagcgagggctatggcgatagcttgactcggctctgtgctgtgctcacctgtgtgttcctgtgcggcgctgctgccaacggcattcgtgtctacctcatgcagtcttcaggtcagagcattgtgaacaggctgcgcacctctctgttctcctccattctaaggcaagaggttgctttctttgacaagacccgcacaggcgaattaattaaccgcctctcctcggataccgcactcctggggcgctccgtgactgagaacctctccgatggcctgagagctggggcccaggcctccgttggtgttggcatgatgttttttgtgtcaccaagtctggccacctttgttctgagtgtggtacctcccatctctgtcctcgctgtgatttatgggcgatatctacggaaactgtccaaagccacacaggactccttggcagaagccacacagctagccgaggagcggattggaaacataagaaccatccgagcttttgggaaggagatgacggaagtggagaagtacaccggccgagtggaccagttgctgcagctggcacagaaggaggccttggcacgagccggcttctttggagcagctgggctctcaggaaacctgattgtgctgtctgtcctgtacaaaggaggcctgctgatgggcagtgcccatatgacagtgggcgagctctcttccttcctcatgtacgctttctgggttggattgagcatcggaggactgagttcattctactccgagctgatgaaaggcctgggtgctggtgggcggctctgggagctgctggagagacagccacggctgccttttaacgaggggatggtgttagatgagaaaaccttccagggtgccctggagttcagaaacgtgcacttcacataccctgctcgcccagaggtgtccgtattccaggatttcagtctttccatcccgtctggatctgtcacagcgctggttggcccaagtggttctgggaaatcaacagtggtttcgctcctgctgcggttgtacgaccctaattctggaacagtcagccttgatggccatgacattcgtcagctaaaccccgtctggctgagatccaagattgggacagtgagtcaggagccagtcctgttctcctgctctgtcgctgagaacattgcctatggagctgacaacctctcctcggtcacagcccagcaggtggagagggccgcagaggtggccaacgctgctgagttcatccgaagcttcccacagggcttcgacactgtggtcggggagaagggcatcctcctgtccggtgggcagaagcagaggattgcaatagccagagccctgctgaagaaccccaaaattcttctccttgatgaagcaaccagtgcactggatgccgaaaatgagcacctggtccaggaggcgcttgaccggctgatggaagggagaactgtgctgatcatagcccaccgcctgtccaccattaagaatgccaactttgttgctgtccttgaccacggaaagatctgtgaacacgggacacatgaagagctgctcctgaagcccaatgggctttacagaaaactgatgaacaagcagagtttcctgtcatataatggagcagagcagttcctggaacctgcacgggcgcctgctcccgcaccagcccctgctcctgcaccagcacctcccagctccggtactaaactcttcaccaaggaaatcccctatgtgaccgagctggagggggacgtaaacggcatgaagtttactatccatggaaagggtaccggtgacgccagcaccgggacaatcaaagcgaaatacatctgcaccaccggcgatctaccggtgccctgggccactcttgtgagcaccctgtcctatggcgtccagtgcttcgcaaagtacccaccggaaatcaaggacttcttcaaatctgccatgccggagggctacgtacaagagaggactatcaccttcgagggcgatggtgtgttcaaaacgcgtgcagaggtcacttttgaaaatggttccgtctacaaccgagtcacgctgacgggccagggattcaaaaaggacggacatatcttgcgtaagaacgtcgcattccagtgtcccccagacatcgtgtacatcctgcccgacactgtgaataacggtatcagagtggagttcaaccaggcatacgatatcgaaggagtaactgagaagctggtgacaaaatgcagccagatgaaccggcctctcgctggctcagcggcagtccacatcccacgctaccaccacctgtcgaaacacaccaaactgtctaaagatcgggacgagaggagagatcatatgtgtctcgtggaggtggtgaaagcggtggacctcgatacgtaccagcaccaccatcaccatcat

SEQ ID NO: 19 - protein, 966 aa, synthetic construct
MSVLTPLLLRGLTGSARRLPVPRAKGSAGSAPEPASPSPAEPAPEKPEPKKPKPKAPKPAEPAPEKPEPKKPKPKAPKPAEPAPEAPEPAAPAPAAPAPAAPAPAAPAPAAPAPAEPAPEAPEPSAPSPAARGRLSAAVGFLAVSSVITMSAPFFLGRIIDVIYTNPSEGYGDSLTRLCAVLTCVFLCGAAANGIRVYLMQSSGQSIVNRLRTSLFSSILRQEVAFFDKTRTGELINRLSSDTALLGRSVTENLSDGLRAGAQASVGVGMMFFVSPSLATFVLSVVPPISVLAVIYGRYLRKLSKATQDSLAEATQLAEERIGNIRTIRAFGKEMTEVEKYTGRVDQLLQLAQKEALARAGFFGAAGLSGNLIVLSVLYKGGLLMGSAHMTVGELSSFLMYAFWVGLSIGGLSSFYSELMKGLGAGGRLWELLERQPRLPFNEGMVLDEKTFQGALEFRNVHFTYPARPEVSVFQDFSLSIPSGSVTALVGPSGSGKSTVVSLLLRLYDPNSGTVSLDGHDIRQLNPVWLRSKIGTVSQEPVLFSCSVAENIAYGADNLSSVTAQQVERAAEVANAAEFIRSFPQGFDTVVGEKGILLSGGQKQRIAIARALLKNPKILLLDEATSALDAENEHLVQEALDRLMEGRTVLIIAHRLSTIKNANFVAVLDHGKICEHGTHEELLLKPNGLYRKLMNKQSFLSYNGAEQFLEPARAPAPAPAPAPAPAPPSSGTKLFTKEIPYVTELEGDVNGMKFTIHGKGTGDASTGTIKAKYICTTGDLPVPWATLVSTLSYGVQCFAKYPPEIKDFFKSAMPEGYVQERTITFEGDGVFKTRAEVTFENGSVYNRVTLTGQGFKKDGHILRKNVAFQCPPDIVYILPDTVNNGIRVEFNQAYDIEGVTEKLVTKCSQMNRPLAGSAAVHIPRYHHLSKHTKLSKDRDERRDHMCLVEVVKAVDLDTYQHHHHHH

SEQ ID NO: 20 - DNA, 2898 bp, synthetic construct
  source 1..2898: mol_type = other DNA
atgtccgtcctgacgccgctgctgctgcggggcttgacaggctcggcccggcggctcccagtgccgcgcgccaagggatcagctggctctgcaccagaaccagcttctccatcacccgctgagcccgctccagagaaaccagagccaaaaaagccaaaacctaaggcccctaagcctgccgagcctgcccctgagaagcctgagcctaagaaacctaagcctaaagcccctaaaccagccgaaccagcccctgaagctcctgaacctgctgcccctgctcctgccgcacctgccccagcagctccagcacccgctgcacccgctccagcagcaccagcacctgcagaacctgcacctgaagcacctgaaccaagtgcaccttcaccagcagctcgcgggagactgtcagctgcagttgggtttctggctgtgtccagtgtcatcaccatgtctgcccccttcttcctgggaaggatcattgatgtcatctataccaacccaagcgagggctatggcgatagcttgactcggctctgtgctgtgctcacctgtgtgttcctgtgcggcgctgctgccaacggcattcgtgtctacctcatgcagtcttcaggtcagagcattgtgaacaggctgcgcacctctctgttctcctccattctaaggcaagaggttgctttctttgacaagacccgcacaggcgaattaattaaccgcctctcctcggataccgcactcctggggcgctccgtgactgagaacctctccgatggcctgagagctggggcccaggcctccgttggtgttggcatgatgttttttgtgtcaccaagtctggccacctttgttctgagtgtggtacctcccatctctgtcctcgctgtgatttatgggcgatatctacggaaactgtccaaagccacacaggactccttggcagaagccacacagctagccgaggagcggattggaaacataagaaccatccgagcttttgggaaggagatgacggaagtggagaagtacaccggccgagtggaccagttgctgcagctggcacagaaggaggccttggcacgagccggcttctttggagcagctgggctctcaggaaacctgattgtgctgtctgtcctgtacaaaggaggcctgctgatgggcagtgcccatatgacagtgggcgagctctcttccttcctcatgtacgctttctgggttggattgagcatcggaggactgagttcattctactccgagctgatgaaaggcctgggtgctggtgggcggctctgggagctgctggagagacagccacggctgccttttaacgaggggatggtgttagatgagaaaaccttccagggtgccctggagttcagaaacgtgcacttcacataccctgctcgcccagaggtgtccgtattccaggatttcagtctttccatcccgtctggatctgtcacagcgctggttggcccaagtggttctgggaaatcaacagtggtttcgctcctgctgcggttgtacgaccctaattctggaacagtcagccttgatggccatgacattcgtcagctaaaccccgtctggctgagatccaagattgggacagtgagtcaggagccagtcctgttctcctgctctgtcgctgagaacattgcctatggagctgacaacctctcctcggtcacagcccagcaggtggagagggccgcagaggtggccaacgctgctgagttcatccgaagcttcccacagggcttcgacactgtggtcggggagaagggcatcctcctgtccggtgggcagaagcagaggattgcaatagccagagccctgctgaagaaccccaaaattcttctccttgatgaagcaaccagtgcactggatgccgaaaatgagcacctggtccaggaggcgcttgaccggctgatggaagggagaactgtgctgatcatagcccaccgcctgtccaccattaagaatgccaactttgttgctgtccttgaccacggaaagatctgtgaacacgggacacatgaagagctgctcctgaagcccaatgggctttacagaaaactgatgaacaagcagagtttcctgtcatataatggagcagagcagttcctggaacctgcacgggcgcctgctcccgcaccagcccctgctcctgcaccagcacctcccagctccggtactaaactcttcaccaaggaaatcccctatgtgaccgagctggagggggacgtaaacggcatgaagtttactatccatggaaagggtaccggtgacgccagcaccgggacaatcaaagcgaaatacatctgcaccaccggcgatctaccggtgccctgggccactcttgtgagcaccctgtcctatggcgtccagtgcttcgcaaagtacccaccggaaatcaaggacttcttcaaatctgccatgccggagggctacgtacaagagaggactatcaccttcgagggcgatggtgtgttcaaaacgcgtgcagaggtcacttttgaaaatggttccgtctacaaccgagtcacgctgacgggccagggattcaaaaaggacggacatatcttgcgtaagaacgtcgcattccagtgtcccccagacatcgtgtacatcctgcccgacactgtgaataacggtatcagagtggagttcaaccaggcatacgatatcgaaggagtaactgagaagctggtgacaaaatgcagccagatgaaccggcctctcgctggctcagcggcagtccacatcccacgctaccaccacctgtcgaaacacaccaaactgtctaaagatcgggacgagaggagagatcatatgtgtctcgtggaggtggtgaaagcggtggacctcgatacgtaccagcaccaccatcaccatcat

SEQ ID NO: 21 - protein, 916 aa, synthetic construct
MSVLTPLLLRGLTGSARRLPVPRAKGSAGSAEAAAQEAAAQEAAAKDAAAKEAAARDAAAREAAAKEAAAKDAAAQEAAARRGRLSAAVGFLAVSSVITMSAPFFLGRIIDVIYTNPSEGYGDSLTRLCAVLTCVFLCGAAANGIRVYLMQSSGQSIVNRLRTSLFSSILRQEVAFFDKTRTGELINRLSSDTALLGRSVTENLSDGLRAGAQASVGVGMMFFVSPSLATFVLSVVPPISVLAVIYGRYLRKLSKATQDSLAEATQLAEERIGNIRTIRAFGKEMTEVEKYTGRVDQLLQLAQKEALARAGFFGAAGLSGNLIVLSVLYKGGLLMGSAHMTVGELSSFLMYAFWVGLSIGGLSSFYSELMKGLGAGGRLWELLERQPRLPFNEGMVLDEKTFQGALEFRNVHFTYPARPEVSVFQDFSLSIPSGSVTALVGPSGSGKSTVVSLLLRLYDPNSGTVSLDGHDIRQLNPVWLRSKIGTVSQEPVLFSCSVAENIAYGADNLSSVTAQQVERAAEVANAAEFIRSFPQGFDTVVGEKGILLSGGQKQRIAIARALLKNPKILLLDEATSALDAENEHLVQEALDRLMEGRTVLIIAHRLSTIKNANFVAVLDHGKICEHGTHEELLLKPNGLYRKLMNKQSFLSYNGAEQFLEPARAPAPAPAPAPAPAPPSSGTKLFTKEIPYVTELEGDVNGMKFTIHGKGTGDASTGTIKAKYICTTGDLPVPWATLVSTLSYGVQCFAKYPPEIKDFFKSAMPEGYVQERTITFEGDGVFKTRAEVTFENGSVYNRVTLTGQGFKKDGHILRKNVAFQCPPDIVYILPDTVNNGIRVEFNQAYDIEGVTEKLVTKCSQMNRPLAGSAAVHIPRYHHLSKHTKLSKDRDERRDHMCLVEVVKAVDLDTYQHHHHHH

SEQ ID NO: 22 - DNA, 2748 bp, synthetic construct
  source 1..2748: mol_type = other DNA
atgtccgtcctgacgccgctgctgctgcggggcttgacaggctcggcccggcggctcccagtgccgcgcgccaagggatcagctggctctgcagaggcagcagcgcaggaagcagctgcacaggaagctgcagctaaagacgccgcagctaaagaagctgctgctcgcgacgctgctgctcgcgaagcagcagctaaggaagcagctgcaaaggacgccgcagcacaggaggcagctgcacggcgcgggagactgtcagctgcagttgggtttctggctgtgtccagtgtcatcaccatgtctgcccccttcttcctgggaaggatcattgatgtcatctataccaacccaagcgagggctatggcgatagcttgactcggctctgtgctgtgctcacctgtgtgttcctgtgcggcgctgctgccaacggcattcgtgtctacctcatgcagtcttcaggtcagagcattgtgaacaggctgcgcacctctctgttctcctccattctaaggcaagaggttgctttctttgacaagacccgcacaggcgaattaattaaccgcctctcctcggataccgcactcctggggcgctccgtgactgagaacctctccgatggcctgagagctggggcccaggcctccgttggtgttggcatgatgttttttgtgtcaccaagtctggccacctttgttctgagtgtggtacctcccatctctgtcctcgctgtgatttatgggcgatatctacggaaactgtccaaagccacacaggactccttggcagaagccacacagctagccgaggagcggattggaaacataagaaccatccgagcttttgggaaggagatgacggaagtggagaagtacaccggccgagtggaccagttgctgcagctggcacagaaggaggccttggcacgagccggcttctttggagcagctgggctctcaggaaacctgattgtgctgtctgtcctgtacaaaggaggcctgctgatgggcagtgcccatatgacagtgggcgagctctcttccttcctcatgtacgctttctgggttggattgagcatcggaggactgagttcattctactccgagctgatgaaaggcctgggtgctggtgggcggctctgggagctgctggagagacagccacggctgccttttaacgaggggatggtgttagatgagaaaaccttccagggtgccctggagttcagaaacgtgcacttcacataccctgctcgcccagaggtgtccgtattccaggatttcagtctttccatcccgtctggatctgtcacagcgctggttggcccaagtggttctgggaaatcaacagtggtttcgctcctgctgcggttgtacgaccctaattctggaacagtcagccttgatggccatgacattcgtcagctaaaccccgtctggctgagatccaagattgggacagtgagtcaggagccagtcctgttctcctgctctgtcgctgagaacattgcctatggagctgacaacctctcctcggtcacagcccagcaggtggagagggccgcagaggtggccaacgctgctgagttcatccgaagcttcccacagggcttcgacactgtggtcggggagaagggcatcctcctgtccggtgggcagaagcagaggattgcaatagccagagccctgctgaagaaccccaaaattcttctccttgatgaagcaaccagtgcactggatgccgaaaatgagcacctggtccaggaggcgcttgaccggctgatggaagggagaactgtgctgatcatagcccaccgcctgtccaccattaagaatgccaactttgttgctgtccttgaccacggaaagatctgtgaacacgggacacatgaagagctgctcctgaagcccaatgggctttacagaaaactgatgaacaagcagagtttcctgtcatataatggagcagagcagttcctggaacctgcacgggcgcctgctcccgcaccagcccctgctcctgcaccagcacctcccagctccggtactaaactcttcaccaaggaaatcccctatgtgaccgagctggagggggacgtaaacggcatgaagtttactatccatggaaagggtaccggtgacgccagcaccgggacaatcaaagcgaaatacatctgcaccaccggcgatctaccggtgccctgggccactcttgtgagcaccctgtcctatggcgtccagtgcttcgcaaagtacccaccggaaatcaaggacttcttcaaatctgccatgccggagggctacgtacaagagaggactatcaccttcgagggcgatggtgtgttcaaaacgcgtgcagaggtcacttttgaaaatggttccgtctacaaccgagtcacgctgacgggccagggattcaaaaaggacggacatatcttgcgtaagaacgtcgcattccagtgtcccccagacatcgtgtacatcctgcccgacactgtgaataacggtatcagagtggagttcaaccaggcatacgatatcgaaggagtaactgagaagctggtgacaaaatgcagccagatgaaccggcctctcgctggctcagcggcagtccacatcccacgctaccaccacctgtcgaaacacaccaaactgtctaaagatcgggacgagaggagagatcatatgtgtctcgtggaggtggtgaaagcggtggacctcgatacgtaccagcaccaccatcaccatcat

SEQ ID NO: 23 - protein, 926 aa, synthetic construct
MSVLTPLLLRGLTGSARRLPVPRAKGSAGSAEAAAQEAAAQEAAAKDAAAKEAAARDAAAREAAAKEAAAKDAAAQEAAAREAAAREAAARRGRLSAAVGFLAVSSVITMSAPFFLGRIIDVIYTNPSEGYGDSLTRLCAVLTCVFLCGAAANGIRVYLMQSSGQSIVNRLRTSLFSSILRQEVAFFDKTRTGELINRLSSDTALLGRSVTENLSDGLRAGAQASVGVGMMFFVSPSLATFVLSVVPPISVLAVIYGRYLRKLSKATQDSLAEATQLAEERIGNIRTIRAFGKEMTEVEKYTGRVDQLLQLAQKEALARAGFFGAAGLSGNLIVLSVLYKGGLLMGSAHMTVGELSSFLMYAFWVGLSIGGLSSFYSELMKGLGAGGRLWELLERQPRLPFNEGMVLDEKTFQGALEFRNVHFTYPARPEVSVFQDFSLSIPSGSVTALVGPSGSGKSTVVSLLLRLYDPNSGTVSLDGHDIRQLNPVWLRSKIGTVSQEPVLFSCSVAENIAYGADNLSSVTAQQVERAAEVANAAEFIRSFPQGFDTVVGEKGILLSGGQKQRIAIARALLKNPKILLLDEATSALDAENEHLVQEALDRLMEGRTVLIIAHRLSTIKNANFVAVLDHGKICEHGTHEELLLKPNGLYRKLMNKQSFLSYNGAEQFLEPARAPAPAPAPAPAPAPPSSGTKLFTKEIPYVTELEGDVNGMKFTIHGKGTGDASTGTIKAKYICTTGDLPVPWATLVSTLSYGVQCFAKYPPEIKDFFKSAMPEGYVQERTITFEGDGVFKTRAEVTFENGSVYNRVTLTGQGFKKDGHILRKNVAFQCPPDIVYILPDTVNNGIRVEFNQAYDIEGVTEKLVTKCSQMNRPLAGSAAVHIPRYHHLSKHTKLSKDRDERRDHMCLVEVVKAVDLDTYQHHHHHH

SEQ ID NO: 24 - DNA, 2778 bp, synthetic construct
  source 1..2778: mol_type = other DNA
atgtccgtcctgacgccgctgctgctgcggggcttgacaggctcggcccggcggctcccagtgccgcgcgccaagggatcagctggctctgcagaggcagcagcgcaggaagcagctgcacaggaagctgcagctaaagacgccgcagctaaagaagctgctgctcgcgacgctgctgctcgcgaagcagcagctaaggaagcagctgcaaaggacgccgcagcacaggaggcagctgcacgggaggcagctgctcgggaagccgctgcccgccgcgggagactgtcagctgcagttgggtttctggctgtgtccagtgtcatcaccatgtctgcccccttcttcctgggaaggatcattgatgtcatctataccaacccaagcgagggctatggcgatagcttgactcggctctgtgctgtgctcacctgtgtgttcctgtgcggcgctgctgccaacggcattcgtgtctacctcatgcagtcttcaggtcagagcattgtgaacaggctgcgcacctctctgttctcctccattctaaggcaagaggttgctttctttgacaagacccgcacaggcgaattaattaaccgcctctcctcggataccgcactcctggggcgctccgtgactgagaacctctccgatggcctgagagctggggcccaggcctccgttggtgttggcatgatgttttttgtgtcaccaagtctggccacctttgttctgagtgtggtacctcccatctctgtcctcgctgtgatttatgggcgatatctacggaaactgtccaaagccacacaggactccttggcagaagccacacagctagccgaggagcggattggaaacataagaaccatccgagcttttgggaaggagatgacggaagtggagaagtacaccggccgagtggaccagttgctgcagctggcacagaaggaggccttggcacgagccggcttctttggagcagctgggctctcaggaaacctgattgtgctgtctgtcctgtacaaaggaggcctgctgatgggcagtgcccatatgacagtgggcgagctctcttccttcctcatgtacgctttctgggttggattgagcatcggaggactgagttcattctactccgagctgatgaaaggcctgggtgctggtgggcggctctgggagctgctggagagacagccacggctgccttttaacgaggggatggtgttagatgagaaaaccttccagggtgccctggagttcagaaacgtgcacttcacataccctgctcgcccagaggtgtccgtattccaggatttcagtctttccatcccgtctggatctgtcacagcgctggttggcccaagtggttctgggaaatcaacagtggtttcgctcctgctgcggttgtacgaccctaattctggaacagtcagccttgatggccatgacattcgtcagctaaaccccgtctggctgagatccaagattgggacagtgagtcaggagccagtcctgttctcctgctctgtcgctgagaacattgcctatggagctgacaacctctcctcggtcacagcccagcaggtggagagggccgcagaggtggccaacgctgctgagttcatccgaagcttcccacagggcttcgacactgtggtcggggagaagggcatcctcctgtccggtgggcagaagcagaggattgcaatagccagagccctgctgaagaaccccaaaattcttctccttgatgaagcaaccagtgcactggatgccgaaaatgagcacctggtccaggaggcgcttgaccggctgatggaagggagaactgtgctgatcatagcccaccgcctgtccaccattaagaatgccaactttgttgctgtccttgaccacggaaagatctgtgaacacgggacacatgaagagctgctcctgaagcccaatgggctttacagaaaactgatgaacaagcagagtttcctgtcatataatggagcagagcagttcctggaacctgcacgggcgcctgctcccgcaccagcccctgctcctgcaccagcacctcccagctccggtactaaactcttcaccaaggaaatcccctatgtgaccgagctggagggggacgtaaacggcatgaagtttactatccatggaaagggtaccggtgacgccagcaccgggacaatcaaagcgaaatacatctgcaccaccggcgatctaccggtgccctgggccactcttgtgagcaccctgtcctatggcgtccagtgcttcgcaaagtacccaccggaaatcaaggacttcttcaaatctgccatgccggagggctacgtacaagagaggactatcaccttcgagggcgatggtgtgttcaaaacgcgtgcagaggtcacttttgaaaatggttccgtctacaaccgagtcacgctgacgggccagggattcaaaaaggacggacatatcttgcgtaagaacgtcgcattccagtgtcccccagacatcgtgtacatcctgcccgacactgtgaataacggtatcagagtggagttcaaccaggcatacgatatcgaaggagtaactgagaagctggtgacaaaatgcagccagatgaaccggcctctcgctggctcagcggcagtccacatcccacgctaccaccacctgtcgaaacacaccaaactgtctaaagatcgggacgagaggagagatcatatgtgtctcgtggaggtggtgaaagcggtggacctcgatacgtaccagcaccaccatcaccatcat

SEQ ID NO: 25 - protein, 936 aa, synthetic construct
MSVLTPLLLRGLTGSARRLPVPRAKGSAGSAEAAAQEAAAQEAAAKDAAAKEAAARDAAAREAAAKEAAAKDAAAQEAAAREAAAREAAARDAAAQEAAARRGRLSAAVGFLAVSSVITMSAPFFLGRIIDVIYTNPSEGYGDSLTRLCAVLTCVFLCGAAANGIRVYLMQSSGQSIVNRLRTSLFSSILRQEVAFFDKTRTGELINRLSSDTALLGRSVTENLSDGLRAGAQASVGVGMMFFVSPSLATFVLSVVPPISVLAVIYGRYLRKLSKATQDSLAEATQLAEERIGNIRTIRAFGKEMTEVEKYTGRVDQLLQLAQKEALARAGFFGAAGLSGNLIVLSVLYKGGLLMGSAHMTVGELSSFLMYAFWVGLSIGGLSSFYSELMKGLGAGGRLWELLERQPRLPFNEGMVLDEKTFQGALEFRNVHFTYPARPEVSVFQDFSLSIPSGSVTALVGPSGSGKSTVVSLLLRLYDPNSGTVSLDGHDIRQLNPVWLRSKIGTVSQEPVLFSCSVAENIAYGADNLSSVTAQQVERAAEVANAAEFIRSFPQGFDTVVGEKGILLSGGQKQRIAIARALLKNPKILLLDEATSALDAENEHLVQEALDRLMEGRTVLIIAHRLSTIKNANFVAVLDHGKICEHGTHEELLLKPNGLYRKLMNKQSFLSYNGAEQFLEPARAPAPAPAPAPAPAPPSSGTKLFTKEIPYVTELEGDVNGMKFTIHGKGTGDASTGTIKAKYICTTGDLPVPWATLVSTLSYGVQCFAKYPPEIKDFFKSAMPEGYVQERTITFEGDGVFKTRAEVTFENGSVYNRVTLTGQGFKKDGHILRKNVAFQCPPDIVYILPDTVNNGIRVEFNQAYDIEGVTEKLVTKCSQMNRPLAGSAAVHIPRYHHLSKHTKLSKDRDERRDHMCLVEVVKAVDLDTYQHHHHHH

SEQ ID NO: 26 - DNA, 2808 bp, synthetic construct
  source 1..2808: mol_type = other DNA
atgtccgtcctgacgccgctgctgctgcggggcttgacaggctcggcccggcggctcccagtgccgcgcgccaagggatcagctggctctgcagaggcagcagcgcaggaagcagctgcacaggaagctgcagctaaagacgccgcagctaaagaagctgctgctcgcgacgctgctgctcgcgaagcagcagctaaggaagcagctgcaaaggacgccgcagcacaggaggcagctgcacgggaggcagctgctcgggaagccgctgcccgcgacgccgctgctcaggaagccgctgcacgacgcgggagactgtcagctgcagttgggtttctggctgtgtccagtgtcatcaccatgtctgcccccttcttcctgggaaggatcattgatgtcatctataccaacccaagcgagggctatggcgatagcttgactcggctctgtgctgtgctcacctgtgtgttcctgtgcggcgctgctgccaacggcattcgtgtctacctcatgcagtcttcaggtcagagcattgtgaacaggctgcgcacctctctgttctcctccattctaaggcaagaggttgctttctttgacaagacccgcacaggcgaattaattaaccgcctctcctcggataccgcactcctggggcgctccgtgactgagaacctctccgatggcctgagagctggggcccaggcctccgttggtgttggcatgatgttttttgtgtcaccaagtctggccacctttgttctgagtgtggtacctcccatctctgtcctcgctgtgatttatgggcgatatctacggaaactgtccaaagccacacaggactccttggcagaagccacacagctagccgaggagcggattggaaacataagaaccatccgagcttttgggaaggagatgacggaagtggagaagtacaccggccgagtggaccagttgctgcagctggcacagaaggaggccttggcacgagccggcttctttggagcagctgggctctcaggaaacctgattgtgctgtctgtcctgtacaaaggaggcctgctgatgggcagtgcccatatgacagtgggcgagctctcttccttcctcatgtacgctttctgggttggattgagcatcggaggactgagttcattctactccgagctgatgaaaggcctgggtgctggtgggcggctctgggagctgctggagagacagccacggctgccttttaacgaggggatggtgttagatgagaaaaccttccagggtgccctggagttcagaaacgtgcacttcacataccctgctcgcccagaggtgtccgtattccaggatttcagtctttccatcccgtctggatctgtcacagcgctggttggcccaagtggttctgggaaatcaacagtggtttcgctcctgctgcggttgtacgaccctaattctggaacagtcagccttgatggccatgacattcgtcagctaaaccccgtctggctgagatccaagattgggacagtgagtcaggagccagtcctgttctcctgctctgtcgctgagaacattgcctatggagctgacaacctctcctcggtcacagcccagcaggtggagagggccgcagaggtggccaacgctgctgagttcatccgaagcttcccacagggcttcgacactgtggtcggggagaagggcatcctcctgtccggtgggcagaagcagaggattgcaatagccagagccctgctgaagaaccccaaaattcttctccttgatgaagcaaccagtgcactggatgccgaaaatgagcacctggtccaggaggcgcttgaccggctgatggaagggagaactgtgctgatcatagcccaccgcctgtccaccattaagaatgccaactttgttgctgtccttgaccacggaaagatctgtgaacacgggacacatgaagagctgctcctgaagcccaatgggctttacagaaaactgatgaacaagcagagtttcctgtcatataatggagcagagcagttcctggaacctgcacgggcgcctgctcccgcaccagcccctgctcctgcaccagcacctcccagctccggtactaaactcttcaccaaggaaatcccctatgtgaccgagctggagggggacgtaaacggcatgaagtttactatccatggaaagggtaccggtgacgccagcaccgggacaatcaaagcgaaatacatctgcaccaccggcgatctaccggtgccctgggccactcttgtgagcaccctgtcctatggcgtccagtgcttcgcaaagtacccaccggaaatcaaggacttcttcaaatctgccatgccggagggctacgtacaagagaggactatcaccttcgagggcgatggtgtgttcaaaacgcgtgcagaggtcacttttgaaaatggttccgtctacaaccgagtcacgctgacgggccagggattcaaaaaggacggacatatcttgcgtaagaacgtcgcattccagtgtcccccagacatcgtgtacatcctgcccgacactgtgaataacggtatcagagtggagttcaaccaggcatacgatatcgaaggagtaactgagaagctggtgacaaaatgcagccagatgaaccggcctctcgctggctcagcggcagtccacatcccacgctaccaccacctgtcgaaacacaccaaactgtctaaagatcgggacgagaggagagatcatatgtgtctcgtggaggtggtgaaagcggtggacctcgatacgtaccagcaccaccatcaccatcat

SEQ ID NO: 27 - protein, 946 aa, synthetic construct
MSVLTPLLLRGLTGSARRLPVPRAKGSAGSAEAAAQEAAAQEAAAKDAAAKEAAARDAAAREAAAKEAAAKDAAAQEAAAREAAAREAAARDAAAQEAAARDAAAQEAAAQRGRLSAAVGFLAVSSVITMSAPFFLGRIIDVIYTNPSEGYGDSLTRLCAVLTCVFLCGAAANGIRVYLMQSSGQSIVNRLRTSLFSSILRQEVAFFDKTRTGELINRLSSDTALLGRSVTENLSDGLRAGAQASVGVGMMFFVSPSLATFVLSVVPPISVLAVIYGRYLRKLSKATQDSLAEATQLAEERIGNIRTIRAFGKEMTEVEKYTGRVDQLLQLAQKEALARAGFFGAAGLSGNLIVLSVLYKGGLLMGSAHMTVGELSSFLMYAFWVGLSIGGLSSFYSELMKGLGAGGRLWELLERQPRLPFNEGMVLDEKTFQGALEFRNVHFTYPARPEVSVFQDFSLSIPSGSVTALVGPSGSGKSTVVSLLLRLYDPNSGTVSLDGHDIRQLNPVWLRSKIGTVSQEPVLFSCSVAENIAYGADNLSSVTAQQVERAAEVANAAEFIRSFPQGFDTVVGEKGILLSGGQKQRIAIARALLKNPKILLLDEATSALDAENEHLVQEALDRLMEGRTVLIIAHRLSTIKNANFVAVLDHGKICEHGTHEELLLKPNGLYRKLMNKQSFLSYNGAEQFLEPARAPAPAPAPAPAPAPPSSGTKLFTKEIPYVTELEGDVNGMKFTIHGKGTGDASTGTIKAKYICTTGDLPVPWATLVSTLSYGVQCFAKYPPEIKDFFKSAMPEGYVQERTITFEGDGVFKTRAEVTFENGSVYNRVTLTGQGFKKDGHILRKNVAFQCPPDIVYILPDTVNNGIRVEFNQAYDIEGVTEKLVTKCSQMNRPLAGSAAVHIPRYHHLSKHTKLSKDRDERRDHMCLVEVVKAVDLDTYQHHHHHH

SEQ ID NO: 28 - DNA, 2838 bp, synthetic construct
  source 1..2838: mol_type = other DNA
atgtccgtcctgacgccgctgctgctgcggggcttgacaggctcggcccggcggctcccagtgccgcgcgccaagggatcagctggctctgcagaggcagcagcgcaggaagcagctgcacaggaagctgcagctaaagacgccgcagctaaagaagctgctgctcgcgacgctgctgctcgcgaagcagcagctaaggaagcagctgcaaaggacgccgcagcacaggaggcagctgcacgggaggcagctgctcgggaagccgctgcccgcgacgccgctgctcaggaagccgctgcacgagatgctgctgcacaggaggccgcagcccagcgcgggagactgtcagctgcagttgggtttctggctgtgtccagtgtcatcaccatgtctgcccccttcttcctgggaaggatcattgatgtcatctataccaacccaagcgagggctatggcgatagcttgactcggctctgtgctgtgctcacctgtgtgttcctgtgcggcgctgctgccaacggcattcgtgtctacctcatgcagtcttcaggtcagagcattgtgaacaggctgcgcacctctctgttctcctccattctaaggcaagaggttgctttctttgacaagacccgcacaggcgaattaattaaccgcctctcctcggataccgcactcctggggcgctccgtgactgagaacctctccgatggcctgagagctggggcccaggcctccgttggtgttggcatgatgttttttgtgtcaccaagtctggccacctttgttctgagtgtggtacctcccatctctgtcctcgctgtgatttatgggcgatatctacggaaactgtccaaagccacacaggactccttggcagaagccacacagctagccgaggagcggattggaaacataagaaccatccgagcttttgggaaggagatgacggaagtggagaagtacaccggccgagtggaccagttgctgcagctggcacagaaggaggccttggcacgagccggcttctttggagcagctgggctctcaggaaacctgattgtgctgtctgtcctgtacaaaggaggcctgctgatgggcagtgcccatatgacagtgggcgagctctcttccttcctcatgtacgctttctgggttggattgagcatcggaggactgagttcattctactccgagctgatgaaaggcctgggtgctggtgggcggctctgggagctgctggagagacagccacggctgccttttaacgaggggatggtgttagatgagaaaaccttccagggtgccctggagttcagaaacgtgcacttcacataccctgctcgcccagaggtgtccgtattccaggatttcagtctttccatcccgtctggatctgtcacagcgctggttggcccaagtggttctgggaaatcaacagtggtttcgctcctgctgcggttgtacgaccctaattctggaacagtcagccttgatggccatgacattcgtcagctaaaccccgtctggctgagatccaagattgggacagtgagtcaggagccagtcctgttctcctgctctgtcgctgagaacattgcctatggagctgacaacctctcctcggtcacagcccagcaggtggagagggccgcagaggtggccaacgctgctgagttcatccgaagcttcccacagggcttcgacactgtggtcggggagaagggcatcctcctgtccggtgggcagaagcagaggattgcaatagccagagccctgctgaagaaccccaaaattcttctccttgatgaagcaaccagtgcactggatgccgaaaatgagcacctggtccaggaggcgcttgaccggctgatggaagggagaactgtgctgatcatagcccaccgcctgtccaccattaagaatgccaactttgttgctgtccttgaccacggaaagatctgtgaacacgggacacatgaagagctgctcctgaagcccaatgggctttacagaaaactgatgaacaagcagagtttcctgtcatataatggagcagagcagttcctggaacctgcacgggcgcctgctcccgcaccagcccctgctcctgcaccagcacctcccagctccggtactaaactcttcaccaaggaaatcccctatgtgaccgagctggagggggacgtaaacggcatgaagtttactatccatggaaagggtaccggtgacgccagcaccgggacaatcaaagcgaaatacatctgcaccaccggcgatctaccggtgccctgggccactcttgtgagcaccctgtcctatggcgtccagtgcttcgcaaagtacccaccggaaatcaaggacttcttcaaatctgccatgccggagggctacgtacaagagaggactatcaccttcgagggcgatggtgtgttcaaaacgcgtgcagaggtcacttttgaaaatggttccgtctacaaccgagtcacgctgacgggccagggattcaaaaaggacggacatatcttgcgtaagaacgtcgcattccagtgtcccccagacatcgtgtacatcctgcccgacactgtgaataacggtatcagagtggagttcaaccaggcatacgatatcgaaggagtaactgagaagctggtgacaaaatgcagccagatgaaccggcctctcgctggctcagcggcagtccacatcccacgctaccaccacctgtcgaaacacaccaaactgtctaaagatcgggacgagaggagagatcatatgtgtctcgtggaggtggtgaaagcggtggacctcgatacgtaccagcaccaccatcaccatcat

SEQ ID NO: 29 - protein, 956 aa, synthetic construct
MSVLTPLLLRGLTGSARRLPVPRAKGSAGSAEAAAQEAAAQEAAAKDAAAKEAAARDAAAREAAAKEAAAKDAAAQEAAAREAAAREAAARDAAAQEAAARDAAAQEAAAQEAAAREAAARRGRLSAAVGFLAVSSVITMSAPFFLGRIIDVIYTNPSEGYGDSLTRLCAVLTCVFLCGAAANGIRVYLMQSSGQSIVNRLRTSLFSSILRQEVAFFDKTRTGELINRLSSDTALLGRSVTENLSDGLRAGAQASVGVGMMFFVSPSLATFVLSVVPPISVLAVIYGRYLRKLSKATQDSLAEATQLAEERIGNIRTIRAFGKEMTEVEKYTGRVDQLLQLAQKEALARAGFFGAAGLSGNLIVLSVLYKGGLLMGSAHMTVGELSSFLMYAFWVGLSIGGLSSFYSELMKGLGAGGRLWELLERQPRLPFNEGMVLDEKTFQGALEFRNVHFTYPARPEVSVFQDFSLSIPSGSVTALVGPSGSGKSTVVSLLLRLYDPNSGTVSLDGHDIRQLNPVWLRSKIGTVSQEPVLFSCSVAENIAYGADNLSSVTAQQVERAAEVANAAEFIRSFPQGFDTVVGEKGILLSGGQKQRIAIARALLKNPKILLLDEATSALDAENEHLVQEALDRLMEGRTVLIIAHRLSTIKNANFVAVLDHGKICEHGTHEELLLKPNGLYRKLMNKQSFLSYNGAEQFLEPARAPAPAPAPAPAPAPPSSGTKLFTKEIPYVTELEGDVNGMKFTIHGKGTGDASTGTIKAKYICTTGDLPVPWATLVSTLSYGVQCFAKYPPEIKDFFKSAMPEGYVQERTITFEGDGVFKTRAEVTFENGSVYNRVTLTGQGFKKDGHILRKNVAFQCPPDIVYILPDTVNNGIRVEFNQAYDIEGVTEKLVTKCSQMNRPLAGSAAVHIPRYHHLSKHTKLSKDRDERRDHMCLVEVVKAVDLDTYQHHHHHH

SEQ ID NO: 30 - DNA, 2868 bp, synthetic construct
  source 1..2868: mol_type = other DNA
atgtccgtcctgacgccgctgctgctgcggggcttgacaggctcggcccggcggctcccagtgccgcgcgccaagggatcagctggctctgcagaggcagcagcgcaggaagcagctgcacaggaagctgcagctaaagacgccgcagctaaagaagctgctgctcgcgacgctgctgctcgcgaagcagcagctaaggaagcagctgcaaaggacgccgcagcacaggaggcagctgcacgggaggcagctgctcgggaagccgctgcccgcgacgccgctgctcaggaagccgctgcacgagatgctgctgcacaggaggccgcagcccaggaggctgcggccagggaagcagctgcacgacgcgggagactgtcagctgcagttgggtttctggctgtgtccagtgtcatcaccatgtctgcccccttcttcctgggaaggatcattgatgtcatctataccaacccaagcgagggctatggcgatagcttgactcggctctgtgctgtgctcacctgtgtgttcctgtgcggcgctgctgccaacggcattcgtgtctacctcatgcagtcttcaggtcagagcattgtgaacaggctgcgcacctctctgttctcctccattctaaggcaagaggttgctttctttgacaagacccgcacaggcgaattaattaaccgcctctcctcggataccgcactcctggggcgctccgtgactgagaacctctccgatggcctgagagctggggcccaggcctccgttggtgttggcatgatgttttttgtgtcaccaagtctggccacctttgttctgagtgtggtacctcccatctctgtcctcgctgtgatttatgggcgatatctacggaaactgtccaaagccacacaggactccttggcagaagccacacagctagccgaggagcggattggaaacataagaaccatccgagcttttgggaaggagatgacggaagtggagaagtacaccggccgagtggaccagttgctgcagctggcacagaaggaggccttggcacgagccggcttctttggagcagctgggctctcaggaaacctgattgtgctgtctgtcctgtacaaaggaggcctgctgatgggcagtgcccatatgacagtgggcgagctctcttccttcctcatgtacgctttctgggttggattgagcatcggaggactgagttcattctactccgagctgatgaaaggcctgggtgctggtgggcggctctgggagctgctggagagacagccacggctgccttttaacgaggggatggtgttagatgagaaaaccttccagggtgccctggagttcagaaacgtgcacttcacataccctgctcgcccagaggtgtccgtattccaggatttcagtctttccatcccgtctggatctgtcacagcgctggttggcccaagtggttctgggaaatcaacagtggtttcgctcctgctgcggttgtacgaccctaattctggaacagtcagccttgatggccatgacattcgtcagctaaaccccgtctggctgagatccaagattgggacagtgagtcaggagccagtcctgttctcctgctctgtcgctgagaacattgcctatggagctgacaacctctcctcggtcacagcccagcaggtggagagggccgcagaggtggccaacgctgctgagttcatccgaagcttcccacagggcttcgacactgtggtcggggagaagggcatcctcctgtccggtgggcagaagcagaggattgcaatagccagagccctgctgaagaaccccaaaattcttctccttgatgaagcaaccagtgcactggatgccgaaaatgagcacctggtccaggaggcgcttgaccggctgatggaagggagaactgtgctgatcatagcccaccgcctgtccaccattaagaatgccaactttgttgctgtccttgaccacggaaagatctgtgaacacgggacacatgaagagctgctcctgaagcccaatgggctttacagaaaactgatgaacaagcagagtttcctgtcatataatggagcagagcagttcctggaacctgcacgggcgcctgctcccgcaccagcccctgctcctgcaccagcacctcccagctccggtactaaactcttcaccaaggaaatcccctatgtgaccgagctggagggggacgtaaacggcatgaagtttactatccatggaaagggtaccggtgacgccagcaccgggacaatcaaagcgaaatacatctgcaccaccggcgatctaccggtgccctgggccactcttgtgagcaccctgtcctatggcgtccagtgcttcgcaaagtacccaccggaaatcaaggacttcttcaaatctgccatgccggagggctacgtacaagagaggactatcaccttcgagggcgatggtgtgttcaaaacgcgtgcagaggtcacttttgaaaatggttccgtctacaaccgagtcacgctgacgggccagggattcaaaaaggacggacatatcttgcgtaagaacgtcgcattccagtgtcccccagacatcgtgtacatcctgcccgacactgtgaataacggtatcagagtggagttcaaccaggcatacgatatcgaaggagtaactgagaagctggtgacaaaatgcagccagatgaaccggcctctcgctggctcagcggcagtccacatcccacgctaccaccacctgtcgaaacacaccaaactgtctaaagatcgggacgagaggagagatcatatgtgtctcgtggaggtggtgaaagcggtggacctcgatacgtaccagcaccaccatcaccatcat

SEQ ID NO: 31 - protein, 966 aa, synthetic construct
MSVLTPLLLRGLTGSARRLPVPRAKGSAGSAEAAAQEAAAQEAAAKDAAAKEAAARDAAAREAAAKEAAAKDAAAQEAAAREAAAREAAARDAAAQEAAARDAAAQEAAAQEAAAREAAARDAAAKEAAARRGRLSAAVGFLAVSSVITMSAPFFLGRIIDVIYTNPSEGYGDSLTRLCAVLTCVFLCGAAANGIRVYLMQSSGQSIVNRLRTSLFSSILRQEVAFFDKTRTGELINRLSSDTALLGRSVTENLSDGLRAGAQASVGVGMMFFVSPSLATFVLSVVPPISVLAVIYGRYLRKLSKATQDSLAEATQLAEERIGNIRTIRAFGKEMTEVEKYTGRVDQLLQLAQKEALARAGFFGAAGLSGNLIVLSVLYKGGLLMGSAHMTVGELSSFLMYAFWVGLSIGGLSSFYSELMKGLGAGGRLWELLERQPRLPFNEGMVLDEKTFQGALEFRNVHFTYPARPEVSVFQDFSLSIPSGSVTALVGPSGSGKSTVVSLLLRLYDPNSGTVSLDGHDIRQLNPVWLRSKIGTVSQEPVLFSCSVAENIAYGADNLSSVTAQQVERAAEVANAAEFIRSFPQGFDTVVGEKGILLSGGQKQRIAIARALLKNPKILLLDEATSALDAENEHLVQEALDRLMEGRTVLIIAHRLSTIKNANFVAVLDHGKICEHGTHEELLLKPNGLYRKLMNKQSFLSYNGAEQFLEPARAPAPAPAPAPAPAPPSSGTKLFTKEIPYVTELEGDVNGMKFTIHGKGTGDASTGTIKAKYICTTGDLPVPWATLVSTLSYGVQCFAKYPPEIKDFFKSAMPEGYVQERTITFEGDGVFKTRAEVTFENGSVYNRVTLTGQGFKKDGHILRKNVAFQCPPDIVYILPDTVNNGIRVEFNQAYDIEGVTEKLVTKCSQMNRPLAGSAAVHIPRYHHLSKHTKLSKDRDERRDHMCLVEVVKAVDLDTYQHHHHHH

SEQ ID NO: 32 - DNA, 2898 bp, synthetic construct
  source 1..2898: mol_type = other DNA
atgtccgtcctgacgccgctgctgctgcggggcttgacaggctcggcccggcggctcccagtgccgcgcgccaagggatcagctggctctgcagaggcagcagcgcaggaagcagctgcacaggaagctgcagctaaagacgccgcagctaaagaagctgctgctcgcgacgctgctgctcgcgaagcagcagctaaggaagcagctgcaaaggacgccgcagcacaggaggcagctgcacgggaggcagctgctcgggaagccgctgcccgcgacgccgctgctcaggaagccgctgcacgagatgctgctgcacaggaggccgcagcccaggaggctgcggccagggaagcagctgcacgagacgcagctgcaaaggaggctgccgcacgtcgcgggagactgtcagctgcagttgggtttctggctgtgtccagtgtcatcaccatgtctgcccccttcttcctgggaaggatcattgatgtcatctataccaacccaagcgagggctatggcgatagcttgactcggctctgtgctgtgctcacctgtgtgttcctgtgcggcgctgctgccaacggcattcgtgtctacctcatgcagtcttcaggtcagagcattgtgaacaggctgcgcacctctctgttctcctccattctaaggcaagaggttgctttctttgacaagacccgcacaggcgaattaattaaccgcctctcctcggataccgcactcctggggcgctccgtgactgagaacctctccgatggcctgagagctggggcccaggcctccgttggtgttggcatgatgttttttgtgtcaccaagtctggccacctttgttctgagtgtggtacctcccatctctgtcctcgctgtgatttatgggcgatatctacggaaactgtccaaagccacacaggactccttggcagaagccacacagctagccgaggagcggattggaaacataagaaccatccgagcttttgggaaggagatgacggaagtggagaagtacaccggccgagtggaccagttgctgcagctggcacagaaggaggccttggcacgagccggcttctttggagcagctgggctctcaggaaacctgattgtgctgtctgtcctgtacaaaggaggcctgctgatgggcagtgcccatatgacagtgggcgagctctcttccttcctcatgtacgctttctgggttggattgagcatcggaggactgagttcattctactccgagctgatgaaaggcctgggtgctggtgggcggctctgggagctgctggagagacagccacggctgccttttaacgaggggatggtgttagatgagaaaaccttccagggtgccctggagttcagaaacgtgcacttcacataccctgctcgcccagaggtgtccgtattccaggatttcagtctttccatcccgtctggatctgtcacagcgctggttggcccaagtggttctgggaaatcaacagtggtttcgctcctgctgcggttgtacgaccctaattctggaacagtcagccttgatggccatgacattcgtcagctaaaccccgtctggctgagatccaagattgggacagtgagtcaggagccagtcctgttctcctgctctgtcgctgagaacattgcctatggagctgacaacctctcctcggtcacagcccagcaggtggagagggccgcagaggtggccaacgctgctgagttcatccgaagcttcccacagggcttcgacactgtggtcggggagaagggcatcctcctgtccggtgggcagaagcagaggattgcaatagccagagccctgctgaagaaccccaaaattcttctccttgatgaagcaaccagtgcactggatgccgaaaatgagcacctggtccaggaggcgcttgaccggctgatggaagggagaactgtgctgatcatagcccaccgcctgtccaccattaagaatgccaactttgttgctgtccttgaccacggaaagatctgtgaacacgggacacatgaagagctgctcctgaagcccaatgggctttacagaaaactgatgaacaagcagagtttcctgtcatataatggagcagagcagttcctggaacctgcacgggcgcctgctcccgcaccagcccctgctcctgcaccagcacctcccagctccggtactaaactcttcaccaaggaaatcccctatgtgaccgagctggagggggacgtaaacggcatgaagtttactatccatggaaagggtaccggtgacgccagcaccgggacaatcaaagcgaaatacatctgcaccaccggcgatctaccggtgccctgggccactcttgtgagcaccctgtcctatggcgtccagtgcttcgcaaagtacccaccggaaatcaaggacttcttcaaatctgccatgccggagggctacgtacaagagaggactatcaccttcgagggcgatggtgtgttcaaaacgcgtgcagaggtcacttttgaaaatggttccgtctacaaccgagtcacgctgacgggccagggattcaaaaaggacggacatatcttgcgtaagaacgtcgcattccagtgtcccccagacatcgtgtacatcctgcccgacactgtgaataacggtatcagagtggagttcaaccaggcatacgatatcgaaggagtaactgagaagctggtgacaaaatgcagccagatgaaccggcctctcgctggctcagcggcagtccacatcccacgctaccaccacctgtcgaaacacaccaaactgtctaaagatcgggacgagaggagagatcatatgtgtctcgtggaggtggtgaaagcggtggacctcgatacgtaccagcaccaccatcaccatcat

SEQ ID NO: 33 - protein, 1066 aa, synthetic construct
MSVLTPLLLRGLTGSARRLPVPRAKGSAGSAEAAAQEAAAQEAAAKDAAAKEAAARDAAAREAAAKEAAAKDAAAQEAAAREAAAREAAARDAAAQEAAARDAAAQEAAAQEAAAREAAARDAAAKEAAAREAAARDAAAREAAAKEAAAKDAAAQEAAAREAAAREAAARDAAAQEAAARDAAAQEAAAQEAAAREAAARDAAAKEAAAREAAAKDAAARDAAAKEAAARRGRLSAAVGFLAVSSVITMSAPFFLGRIIDVIYTNPSEGYGDSLTRLCAVLTCVFLCGAAANGIRVYLMQSSGQSIVNRLRTSLFSSILRQEVAFFDKTRTGELINRLSSDTALLGRSVTENLSDGLRAGAQASVGVGMMFFVSPSLATFVLSVVPPISVLAVIYGRYLRKLSKATQDSLAEATQLAEERIGNIRTIRAFGKEMTEVEKYTGRVDQLLQLAQKEALARAGFFGAAGLSGNLIVLSVLYKGGLLMGSAHMTVGELSSFLMYAFWVGLSIGGLSSFYSELMKGLGAGGRLWELLERQPRLPFNEGMVLDEKTFQGALEFRNVHFTYPARPEVSVFQDFSLSIPSGSVTALVGPSGSGKSTVVSLLLRLYDPNSGTVSLDGHDIRQLNPVWLRSKIGTVSQEPVLFSCSVAENIAYGADNLSSVTAQQVERAAEVANAAEFIRSFPQGFDTVVGEKGILLSGGQKQRIAIARALLKNPKILLLDEATSALDAENEHLVQEALDRLMEGRTVLIIAHRLSTIKNANFVAVLDHGKICEHGTHEELLLKPNGLYRKLMNKQSFLSYNGAEQFLEPARAPAPAPAPAPAPAPPSSGTKLFTKEIPYVTELEGDVNGMKFTIHGKGTGDASTGTIKAKYICTTGDLPVPWATLVSTLSYGVQCFAKYPPEIKDFFKSAMPEGYVQERTITFEGDGVFKTRAEVTFENGSVYNRVTLTGQGFKKDGHILRKNVAFQCPPDIVYILPDTVNNGIRVEFNQAYDIEGVTEKLVTKCSQMNRPLAGSAAVHIPRYHHLSKHTKLSKDRDERRDHMCLVEVVKAVDLDTYQHHHHHH

SEQ ID NO: 34 - DNA, 3198 bp, synthetic construct
  source 1..3198: mol_type = other DNA
atgtccgtcctgacgccgctgctgctgcggggcttgacaggctcggcccggcggctcccagtgccgcgcgccaagggatcagctggctctgcagaggcagcagcgcaggaagcagctgcacaggaagctgcagctaaagacgccgcagctaaagaagctgctgctcgcgacgctgctgctcgcgaagcagcagctaaggaagcagctgcaaaggacgccgcagcacaggaggcagctgcacgggaggcagctgctcgggaagccgctgcccgcgacgccgctgctcaggaagccgctgcacgagatgctgctgcacaggaggccgcagcccaggaggctgcggccagggaagcagctgcacgagacgcagctgcaaaggaggctgccgcacgtgaagctgctgctcgcgacgctgctgctcgcgaagcagcagctaaggaagcagctgcaaaggacgccgcagcacaggaggcagctgcacgggaggcagctgctcgggaagccgctgcccgcgacgccgctgctcaggaagccgctgcacgagatgctgctgcacaggaggccgcagcccaggaggctgcggccagggaagcagctgcacgagacgcagctgcaaaggaggctgccgcacgtgaggctgctgccaaagatgctgctgctcgagatgctgctgctaaggaggccgctgcccgacgcgggagactgtcagctgcagttgggtttctggctgtgtccagtgtcatcaccatgtctgcccccttcttcctgggaaggatcattgatgtcatctataccaacccaagcgagggctatggcgatagcttgactcggctctgtgctgtgctcacctgtgtgttcctgtgcggcgctgctgccaacggcattcgtgtctacctcatgcagtcttcaggtcagagcattgtgaacaggctgcgcacctctctgttctcctccattctaaggcaagaggttgctttctttgacaagacccgcacaggcgaattaattaaccgcctctcctcggataccgcactcctggggcgctccgtgactgagaacctctccgatggcctgagagctggggcccaggcctccgttggtgttggcatgatgttttttgtgtcaccaagtctggccacctttgttctgagtgtggtacctcccatctctgtcctcgctgtgatttatgggcgatatctacggaaactgtccaaagccacacaggactccttggcagaagccacacagctagccgaggagcggattggaaacataagaaccatccgagcttttgggaaggagatgacggaagtggagaagtacaccggccgagtggaccagttgctgcagctggcacagaaggaggccttggcacgagccggcttctttggagcagctgggctctcaggaaacctgattgtgctgtctgtcctgtacaaaggaggcctgctgatgggcagtgcccatatgacagtgggcgagctctcttccttcctcatgtacgctttctgggttggattgagcatcggaggactgagttcattctactccgagctgatgaaaggcctgggtgctggtgggcggctctgggagctgctggagagacagccacggctgccttttaacgaggggatggtgttagatgagaaaaccttccagggtgccctggagttcagaaacgtgcacttcacataccctgctcgcccagaggtgtccgtattccaggatttcagtctttccatcccgtctggatctgtcacagcgctggttggcccaagtggttctgggaaatcaacagtggtttcgctcctgctgcggttgtacgaccctaattctggaacagtcagccttgatggccatgacattcgtcagctaaaccccgtctggctgagatccaagattgggacagtgagtcaggagccagtcctgttctcctgctctgtcgctgagaacattgcctatggagctgacaacctctcctcggtcacagcccagcaggtggagagggccgcagaggtggccaacgctgctgagttcatccgaagcttcccacagggcttcgacactgtggtcggggagaagggcatcctcctgtccggtgggcagaagcagaggattgcaatagccagagccctgctgaagaaccccaaaattcttctccttgatgaagcaaccagtgcactggatgccgaaaatgagcacctggtccaggaggcgcttgaccggctgatggaagggagaactgtgctgatcatagcccaccgcctgtccaccattaagaatgccaactttgttgctgtccttgaccacggaaagatctgtgaacacgggacacatgaagagctgctcctgaagcccaatgggctttacagaaaactgatgaacaagcagagtttcctgtcatataatggagcagagcagttcctggaacctgcacgggcgcctgctcccgcaccagcccctgctcctgcaccagcacctcccagctccggtactaaactcttcaccaaggaaatcccctatgtgaccgagctggagggggacgtaaacggcatgaagtttactatccatggaaagggtaccggtgacgccagcaccgggacaatcaaagcgaaatacatctgcaccaccggcgatctaccggtgccctgggccactcttgtgagcaccctgtcctatggcgtccagtgcttcgcaaagtacccaccggaaatcaaggacttcttcaaatctgccatgccggagggctacgtacaagagaggactatcaccttcgagggcgatggtgtgttcaaaacgcgtgcagaggtcacttttgaaaatggttccgtctacaaccgagtcacgctgacgggccagggattcaaaaaggacggacatatcttgcgtaagaacgtcgcattccagtgtcccccagacatcgtgtacatcctgcccgacactgtgaataacggtatcagagtggagttcaaccaggcatacgatatcgaaggagtaactgagaagctggtgacaaaatgcagccagatgaaccggcctctcgctggctcagcggcagtccacatcccacgctaccaccacctgtcgaaacacaccaaactgtctaaagatcgggacgagaggagagatcatatgtgtctcgtggaggtggtgaaagcggtggacctcgatacgtaccagcaccaccatcaccatcat

SEQ ID NO: 35 - protein, 1166 aa, synthetic construct
MSVLTPLLLRGLTGSARRLPVPRAKGSAGSAEAAAQEAAAQEAAAKDAAAKEAAARDAAAREAAAKEAAAKDAAAQEAAAREAAAREAAARDAAAQEAAARDAAAQEAAAQEAAAREAAARDAAAKEAAAREAAARDAAAREAAAKEAAAKDAAAQEAAAREAAAREAAARDAAAQEAAARDAAAQEAAAQEAAAREAAARDAAAKEAAAREAAAKDAAARDAAAKEAAARDAAAQEAAAREAAAREAAARDAAAQEAAARDAAAQEAAAQEAAAREAAARDAAAKEAAAREAAAKDAAARDAAAKEAAARDAAAQDAAAKDAAAQDAAAKRGRLSAAVGFLAVSSVITMSAPFFLGRIIDVIYTNPSEGYGDSLTRLCAVLTCVFLCGAAANGIRVYLMQSSGQSIVNRLRTSLFSSILRQEVAFFDKTRTGELINRLSSDTALLGRSVTENLSDGLRAGAQASVGVGMMFFVSPSLATFVLSVVPPISVLAVIYGRYLRKLSKATQDSLAEATQLAEERIGNIRTIRAFGKEMTEVEKYTGRVDQLLQLAQKEALARAGFFGAAGLSGNLIVLSVLYKGGLLMGSAHMTVGELSSFLMYAFWVGLSIGGLSSFYSELMKGLGAGGRLWELLERQPRLPFNEGMVLDEKTFQGALEFRNVHFTYPARPEVSVFQDFSLSIPSGSVTALVGPSGSGKSTVVSLLLRLYDPNSGTVSLDGHDIRQLNPVWLRSKIGTVSQEPVLFSCSVAENIAYGADNLSSVTAQQVERAAEVANAAEFIRSFPQGFDTVVGEKGILLSGGQKQRIAIARALLKNPKILLLDEATSALDAENEHLVQEALDRLMEGRTVLIIAHRLSTIKNANFVAVLDHGKICEHGTHEELLLKPNGLYRKLMNKQSFLSYNGAEQFLEPARAPAPAPAPAPAPAPPSSGTKLFTKEIPYVTELEGDVNGMKFTIHGKGTGDASTGTIKAKYICTTGDLPVPWATLVSTLSYGVQCFAKYPPEIKDFFKSAMPEGYVQERTITFEGDGVFKTRAEVTFENGSVYNRVTLTGQGFKKDGHILRKNVAFQCPPDIVYILPDTVNNGIRVEFNQAYDIEGVTEKLVTKCSQMNRPLAGSAAVHIPRYHHLSKHTKLSKDRDERRDHMCLVEVVKAVDLDTYQHHHHHH

SEQ ID NO: 36 - DNA, 3498 bp, synthetic construct
  source 1..3498: mol_type = other DNA
atgtccgtcctgacgccgctgctgctgcggggcttgacaggctcggcccggcggctcccagtgccgcgcgccaagggatcagctggctctgcagaggcagcagcgcaggaagcagctgcacaggaagctgcagctaaagacgccgcagctaaagaagctgctgctcgcgacgctgctgctcgcgaagcagcagctaaggaagcagctgcaaaggacgccgcagcacaggaggcagctgcacgggaggcagctgctcgggaagccgctgcccgcgacgccgctgctcaggaagccgctgcacgagatgctgctgcacaggaggccgcagcccaggaggctgcggccagggaagcagctgcacgagacgcagctgcaaaggaggctgccgcacgtgaagctgctgctcgcgacgctgctgctcgcgaagcagcagctaaggaagcagctgcaaaggacgccgcagcacaggaggcagctgcacgggaggcagctgctcgggaagccgctgcccgcgacgccgctgctcaggaagccgctgcacgagatgctgctgcacaggaggccgcagcccaggaggctgcggccagggaagcagctgcacgagacgcagctgcaaaggaggctgccgcacgtgaggctgctgccaaagatgctgctgctcgagatgctgctgctaaggaggccgctgcccgagacgccgcagcacaggaggcagctgcacgggaggcagctgctcgggaagccgctgcccgcgacgccgctgctcaggaagccgctgcacgagatgctgctgcacaggaggccgcagcccaggaggctgcggccagggaagcagctgcacgagacgcagctgcaaaggaggctgccgcacgtgaggctgctgccaaagatgctgctgctcgagatgctgctgctaaggaggccgctgcccgagatgcagccgcacaggacgcagcagcaaaagacgcagcagctcaggacgctgctgcaaagcgcgggagactgtcagctgcagttgggtttctggctgtgtccagtgtcatcaccatgtctgcccccttcttcctgggaaggatcattgatgtcatctataccaacccaagcgagggctatggcgatagcttgactcggctctgtgctgtgctcacctgtgtgttcctgtgcggcgctgctgccaacggcattcgtgtctacctcatgcagtcttcaggtcagagcattgtgaacaggctgcgcacctctctgttctcctccattctaaggcaagaggttgctttctttgacaagacccgcacaggcgaattaattaaccgcctctcctcggataccgcactcctggggcgctccgtgactgagaacctctccgatggcctgagagctggggcccaggcctccgttggtgttggcatgatgttttttgtgtcaccaagtctggccacctttgttctgagtgtggtacctcccatctctgtcctcgctgtgatttatgggcgatatctacggaaactgtccaaagccacacaggactccttggcagaagccacacagctagccgaggagcggattggaaacataagaaccatccgagcttttgggaaggagatgacggaagtggagaagtacaccggccgagtggaccagttgctgcagctggcacagaaggaggccttggcacgagccggcttctttggagcagctgggctctcaggaaacctgattgtgctgtctgtcctgtacaaaggaggcctgctgatgggcagtgcccatatgacagtgggcgagctctcttccttcctcatgtacgctttctgggttggattgagcatcggaggactgagttcattctactccgagctgatgaaaggcctgggtgctggtgggcggctctgggagctgctggagagacagccacggctgccttttaacgaggggatggtgttagatgagaaaaccttccagggtgccctggagttcagaaacgtgcacttcacataccctgctcgcccagaggtgtccgtattccaggatttcagtctttccatcccgtctggatctgtcacagcgctggttggcccaagtggttctgggaaatcaacagtggtttcgctcctgctgcggttgtacgaccctaattctggaacagtcagccttgatggccatgacattcgtcagctaaaccccgtctggctgagatccaagattgggacagtgagtcaggagccagtcctgttctcctgctctgtcgctgagaacattgcctatggagctgacaacctctcctcggtcacagcccagcaggtggagagggccgcagaggtggccaacgctgctgagttcatccgaagcttcccacagggcttcgacactgtggtcggggagaagggcatcctcctgtccggtgggcagaagcagaggattgcaatagccagagccctgctgaagaaccccaaaattcttctccttgatgaagcaaccagtgcactggatgccgaaaatgagcacctggtccaggaggcgcttgaccggctgatggaagggagaactgtgctgatcatagcccaccgcctgtccaccattaagaatgccaactttgttgctgtccttgaccacggaaagatctgtgaacacgggacacatgaagagctgctcctgaagcccaatgggctttacagaaaactgatgaacaagcagagtttcctgtcatataatggagcagagcagttcctggaacctgcacgggcgcctgctcccgcaccagcccctgctcctgcaccagcacctcccagctccggtactaaactcttcaccaaggaaatcccctatgtgaccgagctggagggggacgtaaacggcatgaagtttactatccatggaaagggtaccggtgacgccagcaccgggacaatcaaagcgaaatacatctgcaccaccggcgatctaccggtgccctgggccactcttgtgagcaccctgtcctatggcgtccagtgcttcgcaaagtacccaccggaaatcaaggacttcttcaaatctgccatgccggagggctacgtacaagagaggactatcaccttcgagggcgatggtgtgttcaaaacgcgtgcagaggtcacttttgaaaatggttccgtctacaaccgagtcacgctgacgggccagggattcaaaaaggacggacatatcttgcgtaagaacgtcgcattccagtgtcccccagacatcgtgtacatcctgcccgacactgtgaataacggtatcagagtggagttcaaccaggcatacgatatcgaaggagtaactgagaagctggtgacaaaatgcagccagatgaaccggcctctcgctggctcagcggcagtccacatcccacgctaccaccacctgtcgaaacacaccaaactgtctaaagatcgggacgagaggagagatcatatgtgtctcgtggaggtggtgaaagcggtggacctcgatacgtaccagcaccaccatcaccatcat

SEQ ID NO: 37 - protein, 1266 aa, synthetic construct
MSVLTPLLLRGLTGSARRLPVPRAKGSAGSAEAAAQEAAAQEAAAKDAAAKEAAARDAAAREAAAKEAAAKDAAAQEAAAREAAAREAAARDAAAQEAAARDAAAQEAAAQEAAAREAAARDAAAKEAAAREAAAQEAAAQEAAAKDAAAKEAAARDAAAREAAAKEAAAKDAAAQEAAAREAAAREAAARDAAAQEAAARDAAAQEAAAQEAAAREAAARDAAAKEAAAREAAARDAAAREAAAKEAAAKDAAAQEAAAREAAAREAAARDAAAQEAAARDAAAQEAAAQEAAAREAAARDAAAKEAAAREAAAKDAAARDAAAKEAAARDAAAQEAAAREAAAREAAARDAAAQEAAARDAAAQEAAAQEAAAREAAARDAAAKEAAAREAAAKDAAARDAAAKEAAARDAAAQDAAAKDAAAQDAAAKRGRLSAAVGFLAVSSVITMSAPFFLGRIIDVIYTNPSEGYGDSLTRLCAVLTCVFLCGAAANGIRVYLMQSSGQSIVNRLRTSLFSSILRQEVAFFDKTRTGELINRLSSDTALLGRSVTENLSDGLRAGAQASVGVGMMFFVSPSLATFVLSVVPPISVLAVIYGRYLRKLSKATQDSLAEATQLAEERIGNIRTIRAFGKEMTEVEKYTGRVDQLLQLAQKEALARAGFFGAAGLSGNLIVLSVLYKGGLLMGSAHMTVGELSSFLMYAFWVGLSIGGLSSFYSELMKGLGAGGRLWELLERQPRLPFNEGMVLDEKTFQGALEFRNVHFTYPARPEVSVFQDFSLSIPSGSVTALVGPSGSGKSTVVSLLLRLYDPNSGTVSLDGHDIRQLNPVWLRSKIGTVSQEPVLFSCSVAENIAYGADNLSSVTAQQVERAAEVANAAEFIRSFPQGFDTVVGEKGILLSGGQKQRIAIARALLKNPKILLLDEATSALDAENEHLVQEALDRLMEGRTVLIIAHRLSTIKNANFVAVLDHGKICEHGTHEELLLKPNGLYRKLMNKQSFLSYNGAEQFLEPARAPAPAPAPAPAPAPPSSGTKLFTKEIPYVTELEGDVNGMKFTIHGKGTGDASTGTIKAKYICTTGDLPVPWATLVSTLSYGVQCFAKYPPEIKDFFKSAMPEGYVQERTITFEGDGVFKTRAEVTFENGSVYNRVTLTGQGFKKDGHILRKNVAFQCPPDIVYILPDTVNNGIRVEFNQAYDIEGVTEKLVTKCSQMNRPLAGSAAVHIPRYHHLSKHTKLSKDRDERRDHMCLVEVVKAVDLDTYQHHHHHH

SEQ ID NO: 38 - DNA, 3798 bp, synthetic construct
  source 1..3798: mol_type = other DNA
atgtccgtcctgacgccgctgctgctgcggggcttgacaggctcggcccggcggctcccagtgccgcgcgccaagggatcagctggctctgcagaggcagcagcgcaggaagcagctgcacaggaagctgcagctaaagacgccgcagctaaagaagctgctgctcgcgacgctgctgctcgcgaagcagcagctaaggaagcagctgcaaaggacgccgcagcacaggaggcagctgcacgggaggcagctgctcgggaagccgctgcccgcgacgccgctgctcaggaagccgctgcacgagatgctgctgcacaggaggccgcagcccaggaggctgcggccagggaagcagctgcacgagacgcagctgcaaaggaggctgccgcacgtgaggcagcagcgcaggaagcagctgcacaggaagctgcagctaaagacgccgcagctaaagaagctgctgctcgcgacgctgctgctcgcgaagcagcagctaaggaagcagctgcaaaggacgccgcagcacaggaggcagctgcacgggaggcagctgctcgggaagccgctgcccgcgacgccgctgctcaggaagccgctgcacgagatgctgctgcacaggaggccgcagcccaggaggctgcggccagggaagcagctgcacgagacgcagctgcaaaggaggctgccgcacgtgaagctgctgctcgcgacgctgctgctcgcgaagcagcagctaaggaagcagctgcaaaggacgccgcagcacaggaggcagctgcacgggaggcagctgctcgggaagccgctgcccgcgacgccgctgctcaggaagccgctgcacgagatgctgctgcacaggaggccgcagcccaggaggctgcggccagggaagcagctgcacgagacgcagctgcaaaggaggctgccgcacgtgaggctgctgccaaagatgctgctgctcgagatgctgctgctaaggaggccgctgcccgagacgccgcagcacaggaggcagctgcacgggaggcagctgctcgggaagccgctgcccgcgacgccgctgctcaggaagccgctgcacgagatgctgctgcacaggaggccgcagcccaggaggctgcggccagggaagcagctgcacgagacgcagctgcaaaggaggctgccgcacgtgaggctgctgccaaagatgctgctgctcgagatgctgctgctaaggaggccgctgcccgagatgcagccgcacaggacgcagcagcaaaagacgcagcagctcaggacgctgctgcaaagcgcgggagactgtcagctgcagttgggtttctggctgtgtccagtgtcatcaccatgtctgcccccttcttcctgggaaggatcattgatgtcatctataccaacccaagcgagggctatggcgatagcttgactcggctctgtgctgtgctcacctgtgtgttcctgtgcggcgctgctgccaacggcattcgtgtctacctcatgcagtcttcaggtcagagcattgtgaacaggctgcgcacctctctgttctcctccattctaaggcaagaggttgctttctttgacaagacccgcacaggcgaattaattaaccgcctctcctcggataccgcactcctggggcgctccgtgactgagaacctctccgatggcctgagagctggggcccaggcctccgttggtgttggcatgatgttttttgtgtcaccaagtctggccacctttgttctgagtgtggtacctcccatctctgtcctcgctgtgatttatgggcgatatctacggaaactgtccaaagccacacaggactccttggcagaagccacacagctagccgaggagcggattggaaacataagaaccatccgagcttttgggaaggagatgacggaagtggagaagtacaccggccgagtggaccagttgctgcagctggcacagaaggaggccttggcacgagccggcttctttggagcagctgggctctcaggaaacctgattgtgctgtctgtcctgtacaaaggaggcctgctgatgggcagtgcccatatgacagtgggcgagctctcttccttcctcatgtacgctttctgggttggattgagcatcggaggactgagttcattctactccgagctgatgaaaggcctgggtgctggtgggcggctctgggagctgctggagagacagccacggctgccttttaacgaggggatggtgttagatgagaaaaccttccagggtgccctggagttcagaaacgtgcacttcacataccctgctcgcccagaggtgtccgtattccaggatttcagtctttccatcccgtctggatctgtcacagcgctggttggcccaagtggttctgggaaatcaacagtggtttcgctcctgctgcggttgtacgaccctaattctggaacagtcagccttgatggccatgacattcgtcagctaaaccccgtctggctgagatccaagattgggacagtgagtcaggagccagtcctgttctcctgctctgtcgctgagaacattgcctatggagctgacaacctctcctcggtcacagcccagcaggtggagagggccgcagaggtggccaacgctgctgagttcatccgaagcttcccacagggcttcgacactgtggtcggggagaagggcatcctcctgtccggtgggcagaagcagaggattgcaatagccagagccctgctgaagaaccccaaaattcttctccttgatgaagcaaccagtgcactggatgccgaaaatgagcacctggtccaggaggcgcttgaccggctgatggaagggagaactgtgctgatcatagcccaccgcctgtccaccattaagaatgccaactttgttgctgtccttgaccacggaaagatctgtgaacacgggacacatgaagagctgctcctgaagcccaatgggctttacagaaaactgatgaacaagcagagtttcctgtcatataatggagcagagcagttcctggaacctgcacgggcgcctgctcccgcaccagcccctgctcctgcaccagcacctcccagctccggtactaaactcttcaccaaggaaatcccctatgtgaccgagctggagggggacgtaaacggcatgaagtttactatccatggaaagggtaccggtgacgccagcaccgggacaatcaaagcgaaatacatctgcaccaccggcgatctaccggtgccctgggccactcttgtgagcaccctgtcctatggcgtccagtgcttcgcaaagtacccaccggaaatcaaggacttcttcaaatctgccatgccggagggctacgtacaagagaggactatcaccttcgagggcgatggtgtgttcaaaacgcgtgcagaggtcacttttgaaaatggttccgtctacaaccgagtcacgctgacgggccagggattcaaaaaggacggacatatcttgcgtaagaacgtcgcattccagtgtcccccagacatcgtgtacatcctgcccgacactgtgaataacggtatcagagtggagttcaaccaggcatacgatatcgaaggagtaactgagaagctggtgacaaaatgcagccagatgaaccggcctctcgctggctcagcggcagtccacatcccacgctaccaccacctgtcgaaacacaccaaactgtctaaagatcgggacgagaggagagatcatatgtgtctcgtggaggtggtgaaagcggtggacctcgatacgtaccagcaccaccatcaccatcat

SEQ ID NO: 39 - protein, 1366 aa, synthetic construct
MSVLTPLLLRGLTGSARRLPVPRAKGSAGSAEAAAQEAAAQEAAAKDAAAKEAAARDAAAREAAAKEAAAKDAAAQEAAAREAAAREAAARDAAAQEAAARDAAAQEAAAQEAAAREAAARDAAAKEAAAREAAARDAAAREAAAKEAAAKDAAAQEAAAREAAAREAAARDAAAQEAAARDAAAQEAAAQEAAAREAAARDAAAKEAAAREAAAKDAAARDAAAKEAAAREAAAQEAAAQEAAAKDAAAKEAAARDAAAREAAAKEAAAKDAAAQEAAAREAAAREAAARDAAAQEAAARDAAAQEAAAQEAAAREAAARDAAAKEAAAREAAARDAAAREAAAKEAAAKDAAAQEAAAREAAAREAAARDAAAQEAAARDAAAQEAAAQEAAAREAAARDAAAKEAAAREAAAKDAAARDAAAKEAAARDAAAQEAAAREAAAREAAARDAAAQEAAARDAAAQEAAAQEAAAREAAARDAAAKEAAAREAAAKDAAARDAAAKEAAARDAAAQDAAAKDAAAQDAAAKRGRLSAAVGFLAVSSVITMSAPFFLGRIIDVIYTNPSEGYGDSLTRLCAVLTCVFLCGAAANGIRVYLMQSSGQSIVNRLRTSLFSSILRQEVAFFDKTRTGELINRLSSDTALLGRSVTENLSDGLRAGAQASVGVGMMFFVSPSLATFVLSVVPPISVLAVIYGRYLRKLSKATQDSLAEATQLAEERIGNIRTIRAFGKEMTEVEKYTGRVDQLLQLAQKEALARAGFFGAAGLSGNLIVLSVLYKGGLLMGSAHMTVGELSSFLMYAFWVGLSIGGLSSFYSELMKGLGAGGRLWELLERQPRLPFNEGMVLDEKTFQGALEFRNVHFTYPARPEVSVFQDFSLSIPSGSVTALVGPSGSGKSTVVSLLLRLYDPNSGTVSLDGHDIRQLNPVWLRSKIGTVSQEPVLFSCSVAENIAYGADNLSSVTAQQVERAAEVANAAEFIRSFPQGFDTVVGEKGILLSGGQKQRIAIARALLKNPKILLLDEATSALDAENEHLVQEALDRLMEGRTVLIIAHRLSTIKNANFVAVLDHGKICEHGTHEELLLKPNGLYRKLMNKQSFLSYNGAEQFLEPARAPAPAPAPAPAPAPPSSGTKLFTKEIPYVTELEGDVNGMKFTIHGKGTGDASTGTIKAKYICTTGDLPVPWATLVSTLSYGVQCFAKYPPEIKDFFKSAMPEGYVQERTITFEGDGVFKTRAEVTFENGSVYNRVTLTGQGFKKDGHILRKNVAFQCPPDIVYILPDTVNNGIRVEFNQAYDIEGVTEKLVTKCSQMNRPLAGSAAVHIPRYHHLSKHTKLSKDRDERRDHMCLVEVVKAVDLDTYQHHHHHH

SEQ ID NO: 40 - DNA, 4098 bp, synthetic construct
  source 1..4098: mol_type = other DNA
atgtccgtcctgacgccgctgctgctgcggggcttgacaggctcggcccggcggctcccagtgccgcgcgccaagggatcagctggctctgcagaggcagcagcgcaggaagcagctgcacaggaagctgcagctaaagacgccgcagctaaagaagctgctgctcgcgacgctgctgctcgcgaagcagcagctaaggaagcagctgcaaaggacgccgcagcacaggaggcagctgcacgggaggcagctgctcgggaagccgctgcccgcgacgccgctgctcaggaagccgctgcacgagatgctgctgcacaggaggccgcagcccaggaggctgcggccagggaagcagctgcacgagacgcagctgcaaaggaggctgccgcacgtgaagctgctgctcgcgacgctgctgctcgcgaagcagcagctaaggaagcagctgcaaaggacgccgcagcacaggaggcagctgcacgggaggcagctgctcgggaagccgctgcccgcgacgccgctgctcaggaagccgctgcacgagatgctgctgcacaggaggccgcagcccaggaggctgcggccagggaagcagctgcacgagacgcagctgcaaaggaggctgccgcacgtgaggctgctgccaaagatgctgctgctcgagatgctgctgctaaggaggccgctgcccgagaggcagcagcgcaggaagcagctgcacaggaagctgcagctaaagacgccgcagctaaagaagctgctgctcgcgacgctgctgctcgcgaagcagcagctaaggaagcagctgcaaaggacgccgcagcacaggaggcagctgcacgggaggcagctgctcgggaagccgctgcccgcgacgccgctgctcaggaagccgctgcacgagatgctgctgcacaggaggccgcagcccaggaggctgcggccagggaagcagctgcacgagacgcagctgcaaaggaggctgccgcacgtgaagctgctgctcgcgacgctgctgctcgcgaagcagcagctaaggaagcagctgcaaaggacgccgcagcacaggaggcagctgcacgggaggcagctgctcgggaagccgctgcccgcgacgccgctgctcaggaagccgctgcacgagatgctgctgcacaggaggccgcagcccaggaggctgcggccagggaagcagctgcacgagacgcagctgcaaaggaggctgccgcacgtgaggctgctgccaaagatgctgctgctcgagatgctgctgctaaggaggccgctgcccgagacgccgcagcacaggaggcagctgcacgggaggcagctgctcgggaagccgctgcccgcgacgccgctgctcaggaagccgctgcacgagatgctgctgcacaggaggccgcagcccaggaggctgcggccagggaagcagctgcacgagacgcagctgcaaaggaggctgccgcacgtgaggctgctgccaaagatgctgctgctcgagatgctgctgctaaggaggccgctgcccgagatgcagccgcacaggacgcagcagcaaaagacgcagcagctcaggacgctgctgcaaagcgcgggagactgtcagctgcagttgggtttctggctgtgtccagtgtcatcaccatgtctgcccccttcttcctgggaaggatcattgatgtcatctataccaacccaagcgagggctatggcgatagcttgactcggctctgtgctgtgctcacctgtgtgttcctgtgcggcgctgctgccaacggcattcgtgtctacctcatgcagtcttcaggtcagagcattgtgaacaggctgcgcacctctctgttctcctccattctaaggcaagaggttgctttctttgacaagacccgcacaggcgaattaattaaccgcctctcctcggataccgcactcctggggcgctccgtgactgagaacctctccgatggcctgagagctggggcccaggcctccgttggtgttggcatgatgttttttgtgtcaccaagtctggccacctttgttctgagtgtggtacctcccatctctgtcctcgctgtgatttatgggcgatatctacggaaactgtccaaagccacacaggactccttggcagaagccacacagctagccgaggagcggattggaaacataagaaccatccgagcttttgggaaggagatgacggaagtggagaagtacaccggccgagtggaccagttgctgcagctggcacagaaggaggccttggcacgagccggcttctttggagcagctgggctctcaggaaacctgattgtgctgtctgtcctgtacaaaggaggcctgctgatgggcagtgcccatatgacagtgggcgagctctcttccttcctcatgtacgctttctgggttggattgagcatcggaggactgagttcattctactccgagctgatgaaaggcctgggtgctggtgggcggctctgggagctgctggagagacagccacggctgccttttaacgaggggatggtgttagatgagaaaaccttccagggtgccctggagttcagaaacgtgcacttcacataccctgctcgcccagaggtgtccgtattccaggatttcagtctttccatcccgtctggatctgtcacagcgctggttggcccaagtggttctgggaaatcaacagtggtttcgctcctgctgcggttgtacgaccctaattctggaacagtcagccttgatggccatgacattcgtcagctaaaccccgtctggctgagatccaagattgggacagtgagtcaggagccagtcctgttctcctgctctgtcgctgagaacattgcctatggagctgacaacctctcctcggtcacagcccagcaggtggagagggccgcagaggtggccaacgctgctgagttcatccgaagcttcccacagggcttcgacactgtggtcggggagaagggcatcctcctgtccggtgggcagaagcagaggattgcaatagccagagccctgctgaagaaccccaaaattcttctccttgatgaagcaaccagtgcactggatgccgaaaatgagcacctggtccaggaggcgcttgaccggctgatggaagggagaactgtgctgatcatagcccaccgcctgtccaccattaagaatgccaactttgttgctgtccttgaccacggaaagatctgtgaacacgggacacatgaagagctgctcctgaagcccaatgggctttacagaaaactgatgaacaagcagagtttcctgtcatataatggagcagagcagttcctggaacctgcacgggcgcctgctcccgcaccagcccctgctcctgcaccagcacctcccagctccggtactaaactcttcaccaaggaaatcccctatgtgaccgagctggagggggacgtaaacggcatgaagtttactatccatggaaagggtaccggtgacgccagcaccgggacaatcaaagcgaaatacatctgcaccaccggcgatctaccggtgccctgggccactcttgtgagcaccctgtcctatggcgtccagtgcttcgcaaagtacccaccggaaatcaaggacttcttcaaatctgccatgccggagggctacgtacaagagaggactatcaccttcgagggcgatggtgtgttcaaaacgcgtgcagaggtcacttttgaaaatggttccgtctacaaccgagtcacgctgacgggccagggattcaaaaaggacggacatatcttgcgtaagaacgtcgcattccagtgtcccccagacatcgtgtacatcctgcccgacactgtgaataacggtatcagagtggagttcaaccaggcatacgatatcgaaggagtaactgagaagctggtgacaaaatgcagccagatgaaccggcctctcgctggctcagcggcagtccacatcccacgctaccaccacctgtcgaaacacaccaaactgtctaaagatcgggacgagaggagagatcatatgtgtctcgtggaggtggtgaaagcggtggacctcgatacgtaccagcaccaccatcaccatcat

SEQ ID NO: 41 - protein, 1466 aa, synthetic construct
MSVLTPLLLRGLTGSARRLPVPRAKGSAGSAEAAAQEAAAQEAAAKDAAAKEAAARDAAAREAAAKEAAAKDAAAQEAAAREAAAREAAARDAAAQEAAARDAAAQEAAAQEAAAREAAARDAAAKEAAAREAAARDAAAREAAAKEAAAKDAAAQEAAAREAAAREAAARDAAAQEAAARDAAAQEAAAQEAAAREAAARDAAAKEAAAREAAAKDAAARDAAAKEAAARDAAAQEAAAREAAAREAAARDAAAQEAAARDAAAQEAAAQEAAAREAAARDAAAKEAAAREAAAKDAAARDAAAKEAAARDAAAQDAAAKDAAAQDAAAKEAAAQEAAAQEAAAKDAAAKEAAARDAAAREAAAKEAAAKDAAAQEAAAREAAAREAAARDAAAQEAAARDAAAQEAAAQEAAAREAAARDAAAKEAAAREAAARDAAAREAAAKEAAAKDAAAQEAAAREAAAREAAARDAAAQEAAARDAAAQEAAAQEAAAREAAARDAAAKEAAAREAAAKDAAARDAAAKEAAARDAAAQEAAAREAAAREAAARDAAAQEAAARDAAAQEAAAQEAAAREAAARDAAAKEAAAREAAAKDAAARDAAAKEAAARDAAAQDAAAKDAAAQDAAAKRGRLSAAVGFLAVSSVITMSAPFFLGRIIDVIYTNPSEGYGDSLTRLCAVLTCVFLCGAAANGIRVYLMQSSGQSIVNRLRTSLFSSILRQEVAFFDKTRTGELINRLSSDTALLGRSVTENLSDGLRAGAQASVGVGMMFFVSPSLATFVLSVVPPISVLAVIYGRYLRKLSKATQDSLAEATQLAEERIGNIRTIRAFGKEMTEVEKYTGRVDQLLQLAQKEALARAGFFGAAGLSGNLIVLSVLYKGGLLMGSAHMTVGELSSFLMYAFWVGLSIGGLSSFYSELMKGLGAGGRLWELLERQPRLPFNEGMVLDEKTFQGALEFRNVHFTYPARPEVSVFQDFSLSIPSGSVTALVGPSGSGKSTVVSLLLRLYDPNSGTVSLDGHDIRQLNPVWLRSKIGTVSQEPVLFSCSVAENIAYGADNLSSVTAQQVERAAEVANAAEFIRSFPQGFDTVVGEKGILLSGGQKQRIAIARALLKNPKILLLDEATSALDAENEHLVQEALDRLMEGRTVLIIAHRLSTIKNANFVAVLDHGKICEHGTHEELLLKPNGLYRKLMNKQSFLSYNGAEQFLEPARAPAPAPAPAPAPAPPSSGTKLFTKEIPYVTELEGDVNGMKFTIHGKGTGDASTGTIKAKYICTTGDLPVPWATLVSTLSYGVQCFAKYPPEIKDFFKSAMPEGYVQERTITFEGDGVFKTRAEVTFENGSVYNRVTLTGQGFKKDGHILRKNVAFQCPPDIVYILPDTVNNGIRVEFNQAYDIEGVTEKLVTKCSQMNRPLAGSAAVHIPRYHHLSKHTKLSKDRDERRDHMCLVEVVKAVDLDTYQHHHHHH

SEQ ID NO: 42 - DNA, 4398 bp, synthetic construct
  source 1..4398: mol_type = other DNA
atgtccgtcctgacgccgctgctgctgcggggcttgacaggctcggcccggcggctcccagtgccgcgcgccaagggatcagctggctctgcagaggcagcagcgcaggaagcagctgcacaggaagctgcagctaaagacgccgcagctaaagaagctgctgctcgcgacgctgctgctcgcgaagcagcagctaaggaagcagctgcaaaggacgccgcagcacaggaggcagctgcacgggaggcagctgctcgggaagccgctgcccgcgacgccgctgctcaggaagccgctgcacgagatgctgctgcacaggaggccgcagcccaggaggctgcggccagggaagcagctgcacgagacgcagctgcaaaggaggctgccgcacgtgaagctgctgctcgcgacgctgctgctcgcgaagcagcagctaaggaagcagctgcaaaggacgccgcagcacaggaggcagctgcacgggaggcagctgctcgggaagccgctgcccgcgacgccgctgctcaggaagccgctgcacgagatgctgctgcacaggaggccgcagcccaggaggctgcggccagggaagcagctgcacgagacgcagctgcaaaggaggctgccgcacgtgaggctgctgccaaagatgctgctgctcgagatgctgctgctaaggaggccgctgcccgagacgccgcagcacaggaggcagctgcacgggaggcagctgctcgggaagccgctgcccgcgacgccgctgctcaggaagccgctgcacgagatgctgctgcacaggaggccgcagcccaggaggctgcggccagggaagcagctgcacgagacgcagctgcaaaggaggctgccgcacgtgaggctgctgccaaagatgctgctgctcgagatgctgctgctaaggaggccgctgcccgagatgcagccgcacaggacgcagcagcaaaagacgcagcagctcaggacgctgctgcaaaggaggcagcagcgcaggaagcagctgcacaggaagctgcagctaaagacgccgcagctaaagaagctgctgctcgcgacgctgctgctcgcgaagcagcagctaaggaagcagctgcaaaggacgccgcagcacaggaggcagctgcacgggaggcagctgctcgggaagccgctgcccgcgacgccgctgctcaggaagccgctgcacgagatgctgctgcacaggaggccgcagcccaggaggctgcggccagggaagcagctgcacgagacgcagctgcaaaggaggctgccgcacgtgaagctgctgctcgcgacgctgctgctcgcgaagcagcagctaaggaagcagctgcaaaggacgccgcagcacaggaggcagctgcacgggaggcagctgctcgggaagccgctgcccgcgacgccgctgctcaggaagccgctgcacgagatgctgctgcacaggaggccgcagcccaggaggctgcggccagggaagcagctgcacgagacgcagctgcaaaggaggctgccgcacgtgaggctgctgccaaagatgctgctgctcgagatgctgctgctaaggaggccgctgcccgagacgccgcagcacaggaggcagctgcacgggaggcagctgctcgggaagccgctgcccgcgacgccgctgctcaggaagccgctgcacgagatgctgctgcacaggaggccgcagcccaggaggctgcggccagggaagcagctgcacgagacgcagctgcaaaggaggctgccgcacgtgaggctgctgccaaagatgctgctgctcgagatgctgctgctaaggaggccgctgcccgagatgcagccgcacaggacgcagcagcaaaagacgcagcagctcaggacgctgctgcaaagcgcgggagactgtcagctgcagttgggtttctggctgtgtccagtgtcatcaccatgtctgcccccttcttcctgggaaggatcattgatgtcatctataccaacccaagcgagggctatggcgatagcttgactcggctctgtgctgtgctcacctgtgtgttcctgtgcggcgctgctgccaacggcattcgtgtctacctcatgcagtcttcaggtcagagcattgtgaacaggctgcgcacctctctgttctcctccattctaaggcaagaggttgctttctttgacaagacccgcacaggcgaattaattaaccgcctctcctcggataccgcactcctggggcgctccgtgactgagaacctctccgatggcctgagagctggggcccaggcctccgttggtgttggcatgatgttttttgtgtcaccaagtctggccacctttgttctgagtgtggtacctcccatctctgtcctcgctgtgatttatgggcgatatctacggaaactgtccaaagccacacaggactccttggcagaagccacacagctagccgaggagcggattggaaacataagaaccatccgagcttttgggaaggagatgacggaagtggagaagtacaccggccgagtggaccagttgctgcagctggcacagaaggaggccttggcacgagccggcttctttggagcagctgggctctcaggaaacctgattgtgctgtctgtcctgtacaaaggaggcctgctgatgggcagtgcccatatgacagtgggcgagctctcttccttcctcatgtacgctttctgggttggattgagcatcggaggactgagttcattctactccgagctgatgaaaggcctgggtgctggtgggcggctctgggagctgctggagagacagccacggctgccttttaacgaggggatggtgttagatgagaaaaccttccagggtgccctggagttcagaaacgtgcacttcacataccctgctcgcccagaggtgtccgtattccaggatttcagtctttccatcccgtctggatctgtcacagcgctggttggcccaagtggttctgggaaatcaacagtggtttcgctcctgctgcggttgtacgaccctaattctggaacagtcagccttgatggccatgacattcgtcagctaaaccccgtctggctgagatccaagattgggacagtgagtcaggagccagtcctgttctcctgctctgtcgctgagaacattgcctatggagctgacaacctctcctcggtcacagcccagcaggtggagagggccgcagaggtggccaacgctgctgagttcatccgaagcttcccacagggcttcgacactgtggtcggggagaagggcatcctcctgtccggtgggcagaagcagaggattgcaatagccagagccctgctgaagaaccccaaaattcttctccttgatgaagcaaccagtgcactggatgccgaaaatgagcacctggtccaggaggcgcttgaccggctgatggaagggagaactgtgctgatcatagcccaccgcctgtccaccattaagaatgccaactttgttgctgtccttgaccacggaaagatctgtgaacacgggacacatgaagagctgctcctgaagcccaatgggctttacagaaaactgatgaacaagcagagtttcctgtcatataatggagcagagcagttcctggaacctgcacgggcgcctgctcccgcaccagcccctgctcctgcaccagcacctcccagctccggtactaaactcttcaccaaggaaatcccctatgtgaccgagctggagggggacgtaaacggcatgaagtttactatccatggaaagggtaccggtgacgccagcaccgggacaatcaaagcgaaatacatctgcaccaccggcgatctaccggtgccctgggccactcttgtgagcaccctgtcctatggcgtccagtgcttcgcaaagtacccaccggaaatcaaggacttcttcaaatctgccatgccggagggctacgtacaagagaggactatcaccttcgagggcgatggtgtgttcaaaacgcgtgcagaggtcacttttgaaaatggttccgtctacaaccgagtcacgctgacgggccagggattcaaaaaggacggacatatcttgcgtaagaacgtcgcattccagtgtcccccagacatcgtgtacatcctgcccgacactgtgaataacggtatcagagtggagttcaaccaggcatacgatatcgaaggagtaactgagaagctggtgacaaaatgcagccagatgaaccggcctctcgctggctcagcggcagtccacatcccacgctaccaccacctgtcgaaacacaccaaactgtctaaagatcgggacgagaggagagatcatatgtgtctcgtggaggtggtgaaagcggtggacctcgatacgtaccagcaccaccatcaccatcat